European Patent Application EP 4 374 922 A2, published May 29, 2024. Title: ANTI-C5 ANTIBODIES AND USES THEREOF. Applicant: REGENERON PHARMACEUTICALS, INC. Application EP, filed June 13, 2017. The sequence listing filed with the application follows.

SEQUENCE LISTING (366 sequences)

SEQ ID NO: 1 - DNA, 357 bp, synthetic construct
  misc_feature 1..357: note = synthetic
  source 1..357: mol_type = other DNA
caggtgcagctggtggagtctgggggaggcgtggtccagcctggaaggtccctgagactctcctgtgtagcgtctggattcaccttcagtagttatggcattcactgggtccgccaggctccaggcaaggggctggagtgggtggcagttatatgggatgatggaaataatataaactattcagactccgtgaagggccgattcatcatctccagagacaattccaggaagacagtgtatctgcaaatgaacagcctgagaggcgaggacacggctgtttattactgtgcgagagatgcccccatagcaccagtccctgactattggggccagggaaccctggtcaccgtctcctca

SEQ ID NO: 2 - protein, 119 aa, synthetic construct
  REGION 1..119: note = synthetic
QVQLVESGGGVVQPGRSLRLSCVASGFTFSSYGIHWVRQAPGKGLEWVAVIWDDGNNINYSDSVKGRFIISRDNSRKTVYLQMNSLRGEDTAVYYCARDAPIAPVPDYWGQGTLVTVSS

SEQ ID NO: 3 - DNA, 24 bp, synthetic construct
  misc_feature 1..24: note = synthetic
  source 1..24: mol_type = other DNA
ggattcaccttcagtagttatggc

SEQ ID NO: 4 - protein, 8 aa, synthetic construct
  REGION 1..8: note = synthetic
GFTFSSYG

SEQ ID NO: 5 - DNA, 24 bp, synthetic construct
  misc_feature 1..24: note = synthetic
  source 1..24: mol_type = other DNA
atatgggatgatggaaataatata

SEQ ID NO: 6 - protein, 8 aa, synthetic construct
  REGION 1..8: note = synthetic
IWDDGNNI

SEQ ID NO: 7 - DNA, 36 bp, synthetic construct
  misc_feature 1..36: note = synthetic
  source 1..36: mol_type = other DNA
gcgagagatgcccccatagcaccagtccctgactat

SEQ ID NO: 8 - protein, 12 aa, synthetic construct
  REGION 1..12: note = synthetic
ARDAPIAPVPDY

SEQ ID NO: 9 - DNA, 321 bp, synthetic construct
  misc_feature 1..321: note = synthetic
  source 1..321: mol_type = other DNA
gacatccagatgacccagtctccttccaccctgtctgcatctgtaggagacagagtcaccatcacttgccgggccagtcagagtattagtagttggttggcctggtatcagcagaaaccagggaaagcccctaagctcctgatctataaggcgtctagtttagacactggggtcccatcaaggttcagcggcagtggatctgggacagagttcactctcaccatcagcagcctgcagcctgatgattttgcaacttattactgccaacagtataatacttattcgtacacttttggcctggggaccaaactggagatcaaa

SEQ ID NO: 10 - protein, 107 aa, synthetic construct
  REGION 1..107: note = synthetic
DIQMTQSPSTLSASVGDRVTITCRASQSISSWLAWYQQKPGKAPKLLIYKASSLDTGVPSRFSGSGSGTEFTLTISSLQPDDFATYYCQQYNTYSYTFGLGTKLEIK

SEQ ID NO: 11 - DNA, 18 bp, synthetic construct
  misc_feature 1..18: note = synthetic
  source 1..18: mol_type = other DNA
cagagtattagtagttgg

SEQ ID NO: 12 - protein, 6 aa, synthetic construct
  REGION 1..6: note = synthetic
QSISSW

SEQ ID NO: 13-14 - skipped (2 entries)

SEQ ID NO: 15 - DNA, 27 bp, synthetic construct
  misc_feature 1..27: note = synthetic
  source 1..27: mol_type = other DNA
caacagtataatacttattcgtacact

SEQ ID NO: 16 - protein, 9 aa, synthetic construct
  REGION 1..9: note = synthetic
QQYNTYSYT

SEQ ID NO: 17 - DNA, 357 bp, synthetic construct
  misc_feature 1..357: note = synthetic
  source 1..357: mol_type = other DNA
caggtgcaactggtggagtctgggggaggcttggtcaagcctggagggtccctgagactctcctgtgcagcttctggattcaccttcagtgactactacatgagctggatccgccaggctccagggaaggggctggagtgggtttcatatattagcagtagtggtaataccataaaatatgcagactctatgaagggccgattcaccatctccagggacaacgccaagaaatcactgtttgtggaaatgaacagcctgagagccgaggacacggccgtgtattactgtgcgaggtataaaagttcgtccgactactttgaccactggggccagggaaccctggtcaccgtctcctca

SEQ ID NO: 18 - protein, 119 aa, synthetic construct
  REGION 1..119: note = synthetic
QVQLVESGGGLVKPGGSLRLSCAASGFTFSDYYMSWIRQAPGKGLEWVSYISSSGNTIKYADSMKGRFTISRDNAKKSLFVEMNSLRAEDTAVYYCARYKSSSDYFDHWGQGTLVTVSS

SEQ ID NO: 19 - DNA, 24 bp, synthetic construct
  misc_feature 1..24: note = synthetic
  source 1..24: mol_type = other DNA
ggattcaccttcagtgactactac

SEQ ID NO: 20 - protein, 8 aa, synthetic construct
  REGION 1..8: note = synthetic
GFTFSDYY

SEQ ID NO: 21 - DNA, 24 bp, synthetic construct
  misc_feature 1..24: note = synthetic
  source 1..24: mol_type = other DNA
attagcagtagtggtaataccata

SEQ ID NO: 22 - protein, 8 aa, synthetic construct
  REGION 1..8: note = synthetic
ISSSGNTI

SEQ ID NO: 23 - DNA, 36 bp, synthetic construct
  misc_feature 1..36: note = synthetic
  source 1..36: mol_type = other DNA
gcgaggtataaaagttcgtccgactactttgaccac

SEQ ID NO: 24 - protein, 12 aa, synthetic construct
  REGION 1..12: note = synthetic
ARYKSSSDYFDH

SEQ ID NO: 25 - DNA, 321 bp, synthetic construct
  misc_feature 1..321: note = synthetic
  source 1..321: mol_type = other DNA
gaaattgtgttgacacagtctccagccaccctgtctttgtctccaggggaaagagccaccctctcctgcagggccagtcagagtgttaggagttacttagcctggtaccaacagaaacctggccaggctcccaggctcctcatctatgatgcatccaacagggccactgccatcccagccaggttcagtggcagtgggtctgggacagacttcactctcaccatcagcagcctagagcctgaagatttagcagtttattactgtcagcagtctggcaactggccgctcactttcggcggagggaccaaggtggagatcaaa

SEQ ID NO: 26 - protein, 107 aa, synthetic construct
  REGION 1..107: note = synthetic
EIVLTQSPATLSLSPGERATLSCRASQSVRSYLAWYQQKPGQAPRLLIYDASNRATAIPARFSGSGSGTDFTLTISSLEPEDLAVYYCQQSGNWPLTFGGGTKVEIK

SEQ ID NO: 27 - DNA, 18 bp, synthetic construct
  misc_feature 1..18: note = synthetic
  source 1..18: mol_type = other DNA
cagagtgttaggagttac

SEQ ID NO: 28 - protein, 6 aa, synthetic construct
  REGION 1..6: note = synthetic
QSVRSY

SEQ ID NO: 29-30 - skipped (2 entries)

SEQ ID NO: 31 - DNA, 27 bp, synthetic construct
  misc_feature 1..27: note = synthetic
  source 1..27: mol_type = other DNA
cagcagtctggcaactggccgctcact

SEQ ID NO: 32 - protein, 9 aa, synthetic construct
  REGION 1..9: note = synthetic
QQSGNWPLT

SEQ ID NO: 33 - DNA, 357 bp, synthetic construct
  misc_feature 1..357: note = synthetic
  source 1..357: mol_type = other DNA
caggtgcagctggtggagtctgggggaggcgtggtccagcctgggaggtccttgagactctcctgtggagcgtctggattcaccttcagtacttatggcatgcactgggtccgccaggctccaggcaaggggctggagtgggtggcagttatctgggatgatggaaataataaatattatgcagactccgtgaagggccgattcaccatctccagagacaattcgaagaacacgctgtatctgcagatgaacagcctgagagccgaggacacggctgtttattactgtgcgagagattcagaggtcgccccagttggggactactggggccagggcaccctggtcaccgtctcctca

SEQ ID NO: 34 - protein, 119 aa, synthetic construct
  REGION 1..119: note = synthetic
QVQLVESGGGVVQPGRSLRLSCGASGFTFSTYGMHWVRQAPGKGLEWVAVIWDDGNNKYYADSVKGRFTISRDNSKNTLYLQMNSLRAEDTAVYYCARDSEVAPVGDYWGQGTLVTVSS

SEQ ID NO: 35 - DNA, 24 bp, synthetic construct
  misc_feature 1..24: note = synthetic
  source 1..24: mol_type = other DNA
ggattcaccttcagtacttatggc

SEQ ID NO: 36 - protein, 8 aa, synthetic construct
  REGION 1..8: note = synthetic
GFTFSTYG

SEQ ID NO: 37 - DNA, 24 bp, synthetic construct
  misc_feature 1..24: note = synthetic
  source 1..24: mol_type = other DNA
atctgggatgatggaaataataaa

SEQ ID NO: 38 - protein, 8 aa, synthetic construct
  REGION 1..8: note = synthetic
IWDDGNNK

SEQ ID NO: 39 - DNA, 36 bp, synthetic construct
  misc_feature 1..36: note = synthetic
  source 1..36: mol_type = other DNA
gcgagagattcagaggtcgccccagttggggactac

SEQ ID NO: 40 - protein, 12 aa, synthetic construct
  REGION 1..12: note = synthetic
ARDSEVAPVGDY

SEQ ID NO: 41 - DNA, 321 bp, synthetic construct
  misc_feature 1..321: note = synthetic
  source 1..321: mol_type = other DNA
gacatccagatgacccagtctccttccaccctgtctgcatctgtaggagacagagtcactatcatttgccgggccagtcagagtattaacaggtggttggcctggtatcagcagaaaccagggaaggcccctaaactcctgatctataaggcgtctagtttagaaagtggggtcccatcaaggttcagcggcagtggatctgggacagaattcactctcaccatcagcagcctgcagcctgatgattttgcagcttattactgccaacagtataatgattattcgtacacttttggccaggggaccaagctggagatcaaa

SEQ ID NO: 42 - protein, 107 aa, synthetic construct
  REGION 1..107: note = synthetic
DIQMTQSPSTLSASVGDRVTIICRASQSINRWLAWYQQKPGKAPKLLIYKASSLESGVPSRFSGSGSGTEFTLTISSLQPDDFAAYYCQQYNDYSYTFGQGTKLEIK

SEQ ID NO: 43 - DNA, 18 bp, synthetic construct
  misc_feature 1..18: note = synthetic
  source 1..18: mol_type = other DNA
cagagtattaacaggtgg

SEQ ID NO: 44 - protein, 6 aa, synthetic construct
  REGION 1..6: note = synthetic
QSINRW

SEQ ID NO: 45-46 - skipped (2 entries)

SEQ ID NO: 47 - DNA, 27 bp, synthetic construct
  misc_feature 1..27: note = synthetic
  source 1..27: mol_type = other DNA
caacagtataatgattattcgtacact

SEQ ID NO: 48 - protein, 9 aa, synthetic construct
  REGION 1..9: note = synthetic
QQYNDYSYT

SEQ ID NO: 49 - DNA, 366 bp, synthetic construct
  misc_feature 1..366: note = synthetic
  source 1..366: mol_type = other DNA
gaggtgcagctggtggagtctgggggagacttggtccagcctggagggtccctgagactctcctgtgcagcctctggattcaccttcagtgaccactatatggactgggtccgccaggctccagggaaggggctggactggattggccgtattagaaacaaagctaacgcttataacacagaatacgccgcgtctgtgagaggcagattcaccatctcaagagatgattcacagaatttactgtatctgcaaatgaacagcctgaaaaccgatgacacggccgtatattattgtgttagagtctggaactacgcctacttcgctatggacgtctggggccaagggaccacggtcaccgtctcctca

SEQ ID NO: 50 - protein, 122 aa, synthetic construct
  REGION 1..122: note = synthetic
EVQLVESGGDLVQPGGSLRLSCAASGFTFSDHYMDWVRQAPGKGLDWIGRIRNKANAYNTEYAASVRGRFTISRDDSQNLLYLQMNSLKTDDTAVYYCVRVWNYAYFAMDVWGQGTTVTVSS

SEQ ID NO: 51 - DNA, 24 bp, synthetic construct
  misc_feature 1..24: note = synthetic
  source 1..24: mol_type = other DNA
ggattcaccttcagtgaccactat

SEQ ID NO: 52 - protein, 8 aa, synthetic construct
  REGION 1..8: note = synthetic
GFTFSDHY

SEQ ID NO: 53 - DNA, 30 bp, synthetic construct
  misc_feature 1..30: note = synthetic
  source 1..30: mol_type = other DNA
attagaaacaaagctaacgcttataacaca

SEQ ID NO: 54 - protein, 10 aa, synthetic construct
  REGION 1..10: note = synthetic
IRNKANAYNT

SEQ ID NO: 55 - DNA, 39 bp, synthetic construct
  misc_feature 1..39: note = synthetic
  source 1..39: mol_type = other DNA
gttagagtctggaactacgcctacttcgctatggacgtc

SEQ ID NO: 56 - protein, 13 aa, synthetic construct
  REGION 1..13: note = synthetic
VRVWNYAYFAMDV

SEQ ID NO: 57 - DNA, 321 bp, synthetic construct
  misc_feature 1..321: note = synthetic
  source 1..321: mol_type = other DNA
gacatccagatgacccagtctccatcctccctatctgcatctgtgggagacagagtcaccatcacttgccggtcaagtcagaacattggaatctttttaaactggtatcaacaaaaaccaggggaagcccctaacctcctgatctccgctgcatccagtttacacagtggggtcccttcaaggttcagtggcagtgggtctgggacagatttcactctcaccatcggcagtctgcagcctgaagattttgcgacttactactgtcaacagacgtacaataccatattcactttcggccctgggaccaaagtggatatcaaa

SEQ ID NO: 58 - protein, 107 aa, synthetic construct
  REGION 1..107: note = synthetic
DIQMTQSPSSLSASVGDRVTITCRSSQNIGIFLNWYQQKPGEAPNLLISAASSLHSGVPSRFSGSGSGTDFTLTIGSLQPEDFATYYCQQTYNTIFTFGPGTKVDIK

SEQ ID NO: 59 - DNA, 18 bp, synthetic construct
  misc_feature 1..18: note = synthetic
  source 1..18: mol_type = other DNA
cagaacattggaatcttt

SEQ ID NO: 60 - protein, 6 aa, synthetic construct
  REGION 1..6: note = synthetic
QNIGIF

SEQ ID NO: 61-62 - skipped (2 entries)

SEQ ID NO: 63 - DNA, 27 bp, synthetic construct
  misc_feature 1..27: note = synthetic
  source 1..27: mol_type = other DNA
caacagacgtacaataccatattcact

SEQ ID NO: 64 - protein, 9 aa, synthetic construct
  REGION 1..9: note = synthetic
QQTYNTIFT

SEQ ID NO: 65 - DNA, 363 bp, synthetic construct
  misc_feature 1..363: note = synthetic
  source 1..363: mol_type = other DNA
gaggtgcagctggtggagtctgggggagacttggtacagcctggggggtccctgagactctcctgtgcagcctctggattcacctttagcagctatgccatgaactgggtccgccagggtccagggaagggactggagtgggtctcagctattagtggtcgtggtgatagtacatactacgcagactccgtgaagggccggctcaccatctccagagacaattccaagaacacgctgtatctgcaaatgaacagcctgagagccgaggacacggccgtatattactgtgtgaaagagggggagcaactcgtctactggtacttcgatctctggggccgtggcaccctggtcaccgtctcctca

SEQ ID NO: 66 - protein, 121 aa, synthetic construct
  REGION 1..121: note = synthetic
EVQLVESGGDLVQPGGSLRLSCAASGFTFSSYAMNWVRQGPGKGLEWVSAISGRGDSTYYADSVKGRLTISRDNSKNTLYLQMNSLRAEDTAVYYCVKEGEQLVYWYFDLWGRGTLVTVSS

SEQ ID NO: 67 - DNA, 24 bp, synthetic construct
  misc_feature 1..24: note = synthetic
  source 1..24: mol_type = other DNA
ggattcacctttagcagctatgcc

SEQ ID NO: 68 - protein, 8 aa, synthetic construct
  REGION 1..8: note = synthetic
GFTFSSYA

SEQ ID NO: 69 - DNA, 24 bp, synthetic construct
  misc_feature 1..24: note = synthetic
  source 1..24: mol_type = other DNA
attagtggtcgtggtgatagtaca

SEQ ID NO: 70 - protein, 8 aa, synthetic construct
  REGION 1..8: note = synthetic
ISGRGDST

SEQ ID NO: 71 - DNA, 42 bp, synthetic construct
  misc_feature 1..42: note = synthetic
  source 1..42: mol_type = other DNA
gtgaaagagggggagcaactcgtctactggtacttcgatctc

SEQ ID NO: 72 - protein, 14 aa, synthetic construct
  REGION 1..14: note = synthetic
VKEGEQLVYWYFDL

SEQ ID NO: 73 - DNA, 321 bp, synthetic construct
  misc_feature 1..321: note = synthetic
  source 1..321: mol_type = other DNA
gacatccagatgacccagtctccatcctccctgtctgcatctgtaggagacagagtcaccatcacttgccgggcaagtcagaccattagcaactttttacattggtatcagcagaaaccagggaaagcccctaagctcctgatctatgctgcatccagtttgcaaagtggggtcccatcaaggttcagtggcagtggatctgggacagatttcactctcaccatcagcagtctgcaacctgaagatttttcaacttacttctgtcaacagagttacactaccccgctcactttcggcggagggaccaaggtggagatcaaa

SEQ ID NO: 74 - protein, 107 aa, synthetic construct
  REGION 1..107: note = synthetic
DIQMTQSPSSLSASVGDRVTITCRASQTISNFLHWYQQKPGKAPKLLIYAASSLQSGVPSRFSGSGSGTDFTLTISSLQPEDFSTYFCQQSYTTPLTFGGGTKVEIK

SEQ ID NO: 75 - DNA, 18 bp, synthetic construct
  misc_feature 1..18: note = synthetic
  source 1..18: mol_type = other DNA
cagaccattagcaacttt

SEQ ID NO: 76 - protein, 6 aa, synthetic construct
  REGION 1..6: note = synthetic
QTISNF

SEQ ID NO: 77-78 - skipped (2 entries)

SEQ ID NO: 79 - DNA, 27 bp, synthetic construct
  misc_feature 1..27: note = synthetic
  source 1..27: mol_type = other DNA
caacagagttacactaccccgctcact

SEQ ID NO: 80 - protein, 9 aa, synthetic construct
  REGION 1..9: note = synthetic
QQSYTTPLT

SEQ ID NO: 81 - DNA, 363 bp, synthetic construct
  misc_feature 1..363: note = synthetic
  source 1..363: mol_type = other DNA
gaggtgcagctggtggagtctgggggaggcttggtgaggtcgggggggtccctgagactctcctgtgcagcctctggattcacctttaacagatatgccatgacctgggtccgccaggctccagggaaggggctggagtgggtctcagctataagtggtagtggtagcagcacatactacacagactccgtgaaaggccggttcaccatctccagagacaattccaagaattcggtggatctgcaaatgcacagcctgagagtcgaagacacggccatatattattgtgcgagagggactacagtcactacggggtacggtatggacgtctggggccaagggaccacggtcaccgtctcctca

SEQ ID NO: 82 - protein, 121 aa, synthetic construct
  REGION 1..121: note = synthetic
EVQLVESGGGLVRSGGSLRLSCAASGFTFNRYAMTWVRQAPGKGLEWVSAISGSGSSTYYTDSVKGRFTISRDNSKNSVDLQMHSLRVEDTAIYYCARGTTVTTGYGMDVWGQGTTVTVSS

SEQ ID NO: 83 - DNA, 24 bp, synthetic construct
  misc_feature 1..24: note = synthetic
  source 1..24: mol_type = other DNA
ggattcacctttaacagatatgcc

SEQ ID NO: 84 - protein, 8 aa, synthetic construct
  REGION 1..8: note = synthetic
GFTFNRYA

SEQ ID NO: 85 - DNA, 24 bp, synthetic construct
  misc_feature 1..24: note = synthetic
  source 1..24: mol_type = other DNA
ataagtggtagtggtagcagcaca

SEQ ID NO: 86 - protein, 8 aa, synthetic construct
  REGION 1..8: note = synthetic
ISGSGSST

SEQ ID NO: 87 - DNA, 42 bp, synthetic construct
  misc_feature 1..42: note = synthetic
  source 1..42: mol_type = other DNA
gcgagagggactacagtcactacggggtacggtatggacgtc

SEQ ID NO: 88 - protein, 14 aa, synthetic construct
  REGION 1..14: note = synthetic
ARGTTVTTGYGMDV

SEQ ID NO: 89 - DNA, 321 bp, synthetic construct
  misc_feature 1..321: note = synthetic
  source 1..321: mol_type = other DNA
gacatccagatgacccagtctccatcctccctgtctgcatctgtaggagacagagtcaccttcacttgccaggcgagtcaggacattaccaattctttaaattggtatcaacagaaacctgggagagcccctaagctcctgatctacgatgcatcgtatttgaaggcaggggtcccatcaagattcagtggaagtggatctgggacagattttactttcaccatcagcagcctgcagcctgaagatattgcaacatattactgtcaacaatatgatgatctcccatacacttttggccaggggaccaagctggagatcaaa

SEQ ID NO: 90 - protein, 107 aa, synthetic construct
  REGION 1..107: note = synthetic
DIQMTQSPSSLSASVGDRVTFTCQASQDITNSLNWYQQKPGRAPKLLIYDASYLKAGVPSRFSGSGSGTDFTFTISSLQPEDIATYYCQQYDDLPYTFGQGTKLEIK

SEQ ID NO: 91 - DNA, 18 bp, synthetic construct
  misc_feature 1..18: note = synthetic
  source 1..18: mol_type = other DNA
caggacattaccaattct

SEQ ID NO: 92 - protein, 6 aa, synthetic construct
  REGION 1..6: note = synthetic
QDITNS

SEQ ID NO: 93-94 - skipped (2 entries)

SEQ ID NO: 95 - DNA, 27 bp, synthetic construct
  misc_feature 1..27: note = synthetic
  source 1..27: mol_type = other DNA
caacaatatgatgatctcccatacact

SEQ ID NO: 96 - protein, 9 aa, synthetic construct
  REGION 1..9: note = synthetic
QQYDDLPYT

SEQ ID NO: 97 - DNA, 360 bp, synthetic construct
  misc_feature 1..360: note = synthetic
  source 1..360: mol_type = other DNA
caggtgcagctgcaggagtcgggcccaggactggtgaagccttcggagaccctgtccctcacctgcactgtctctggtgactccgtcagtagttcctactggacctggatccggcagcccccagggaagggactggagtggattggctatatctattacagtgggagttccaactacaacccctccctcaagagtcgagccaccatttcagtagacacgtccaagaaccagttctccctgaagctgagttctgtgaccgctgcggacacggccgtatattactgtgcgagagaagggaacgtggatacaactatgatatttgactactggggccagggaaccctggtcaccgtctcctca

SEQ ID NO: 98 - protein, 120 aa, synthetic construct
  REGION 1..120: note = synthetic
QVQLQESGPGLVKPSETLSLTCTVSGDSVSSSYWTWIRQPPGKGLEWIGYIYYSGSSNYNPSLKSRATISVDTSKNQFSLKLSSVTAADTAVYYCAREGNVDTTMIFDYWGQGTLVTVSS

SEQ ID NO: 99 - DNA, 24 bp, synthetic construct
  misc_feature 1..24: note = synthetic
  source 1..24: mol_type = other DNA
ggtgactccgtcagtagttcctac

SEQ ID NO: 100 - protein, 8 aa, synthetic construct
  REGION 1..8: note = synthetic
GDSVSSSY

SEQ ID NO: 101 - DNA, 21 bp, synthetic construct
  misc_feature 1..21: note = synthetic
  source 1..21: mol_type = other DNA
atctattacagtgggagttcc

SEQ ID NO: 102 - protein, 7 aa, synthetic construct
  REGION 1..7: note = synthetic
IYYSGSS

SEQ ID NO: 103 - DNA, 42 bp, synthetic construct
  misc_feature 1..42: note = synthetic
  source 1..42: mol_type = other DNA
gcgagagaagggaacgtggatacaactatgatatttgactac

SEQ ID NO: 104 - protein, 14 aa, synthetic construct
  REGION 1..14: note = synthetic
AREGNVDTTMIFDY

SEQ ID NO: 105 - DNA, 321 bp, synthetic construct
  misc_feature 1..321: note = synthetic
  source 1..321: mol_type = other DNA
gccatccagatgacccagtctccatcctccctgtctgcatctgtaggagacagagtcaccatcacttgccgggcaagtcagggcattagaaatgatttaggctggtatcaacagaaaccagggaaagcccctaaactcctgatctatgctgcatccagtttacaaagtggggtcccatcgaggttcgccggccgtggatctggcacagatttcactctcaccatcagcagcctgcagcctgaagattttgcaacttattactgtctacaagatttcaattacccgtggacgttcggccaagggaccaaggtggaaatcaaa

SEQ ID NO: 106 - protein, 107 aa, synthetic construct
  REGION 1..107: note = synthetic
AIQMTQSPSSLSASVGDRVTITCRASQGIRNDLGWYQQKPGKAPKLLIYAASSLQSGVPSRFAGRGSGTDFTLTISSLQPEDFATYYCLQDFNYPWTFGQGTKVEIK

SEQ ID NO: 107 - DNA, 18 bp, synthetic construct
  misc_feature 1..18: note = synthetic
  source 1..18: mol_type = other DNA
cagggcattagaaatgat

SEQ ID NO: 108 - protein, 6 aa, synthetic construct
  REGION 1..6: note = synthetic
QGIRND

SEQ ID NO: 109-110 - skipped (2 entries)

SEQ ID NO: 111 - DNA, 27 bp, synthetic construct
  misc_feature 1..27: note = synthetic
  source 1..27: mol_type = other DNA
ctacaagatttcaattacccgtggacg

SEQ ID NO: 112 - protein, 9 aa, synthetic construct
  REGION 1..9: note = synthetic
LQDFNYPWT

SEQ ID NO: 113 - DNA, 321 bp, synthetic construct
  misc_feature 1..321: note = synthetic
  source 1..321: mol_type = other DNA
gccatccagatgacccagtctccatcctccctgtctgcatctgtaggagacagagtcaccatcacttgccgggcaagtcagggcattagaaatgatttaggctggtatcaacagaaaccagggaaagcccctaaactcctgatctatgctgcatccagtttacaaagtggggtcccatcgaggttcgccggccgtggatctggcacagatttcactctcaccatcagcagcctgcagcctgaagattttgcaacttattactgtcatcaagatttcaattacccgtggacgttcggccaagggaccaaggtggaaatcaaa

SEQ ID NO: 114 - protein, 107 aa, synthetic construct
  REGION 1..107: note = synthetic
AIQMTQSPSSLSASVGDRVTITCRASQGIRNDLGWYQQKPGKAPKLLIYAASSLQSGVPSRFAGRGSGTDFTLTISSLQPEDFATYYCHQDFNYPWTFGQGTKVEIK

SEQ ID NO: 115 - DNA, 18 bp, synthetic construct
  misc_feature 1..18: note = synthetic
  source 1..18: mol_type = other DNA
cagggcattagaaatgat

SEQ ID NO: 116 - protein, 6 aa, synthetic construct
  REGION 1..6: note = synthetic
QGIRND

SEQ ID NO: 117-118 - skipped (2 entries)

SEQ ID NO: 119 - DNA, 27 bp, synthetic construct
  misc_feature 1..27: note = synthetic
  source 1..27: mol_type = other DNA
catcaagatttcaattacccgtggacg

SEQ ID NO: 120 - protein, 9 aa, synthetic construct
  REGION 1..9: note = synthetic
HQDFNYPWT

SEQ ID NO: 121 - DNA, 360 bp, synthetic construct
  misc_feature 1..360: note = synthetic
  source 1..360: mol_type = other DNA
caggtgcagctgcaggagtcgggcccaggactggtgaagccttcggagaccctgtccctcacctgcactgtctctggtgactccgtcagtagttcctactggacctggatccggcagcccccagggaagggactggagtggattggctatatctattacagtgggagttccaactacaacccctccctcaagagtcgagccaccatttcagtagacacgtccaagaaccagttctccctgaagctgagttctgtgaccgctgcggacacggccgtatattactgtgcgagagaacataacgtggatacaactatgatatttgactactggggccagggaaccctggtcaccgtctcctca

SEQ ID NO: 122 - protein, 120 aa, synthetic construct
  REGION 1..120: note = synthetic
QVQLQESGPGLVKPSETLSLTCTVSGDSVSSSYWTWIRQPPGKGLEWIGYIYYSGSSNYNPSLKSRATISVDTSKNQFSLKLSSVTAADTAVYYCAREHNVDTTMIFDYWGQGTLVTVSS

SEQ ID NO: 123 - DNA, 24 bp, synthetic construct
  misc_feature 1..24: note = synthetic
  source 1..24: mol_type = other DNA
ggtgactccgtcagtagttcctac

SEQ ID NO: 124 - protein, 8 aa, synthetic construct
  REGION 1..8: note = synthetic
GDSVSSSY

SEQ ID NO: 125 - DNA, 21 bp, synthetic construct
  misc_feature 1..21: note = synthetic
  source 1..21: mol_type = other DNA
atctattacagtgggagttcc

SEQ ID NO: 126 - protein, 7 aa, synthetic construct
  REGION 1..7: note = synthetic
IYYSGSS

SEQ ID NO: 127 - DNA, 42 bp, synthetic construct
  misc_feature 1..42: note = synthetic
  source 1..42: mol_type = other DNA
gcgagagaacataacgtggatacaactatgatatttgactac

SEQ ID NO: 128 - protein, 14 aa, synthetic construct
  REGION 1..14: note = synthetic
AREHNVDTTMIFDY

SEQ ID NO: 129 - DNA, 321 bp, synthetic construct
  misc_feature 1..321: note = synthetic
  source 1..321: mol_type = other DNA
gccatccagatgacccagtctccatcctccctgtctgcatctgtaggagacagagtcaccatcacttgccgggcaagtcagggcattagaaatgatttaggctggtatcaacagaaaccagggaaagcccctaaactcctgatctatgctgcatccagtttacaaagtggggtcccatcgaggttcgccggccgtggatctggcacagatttcactctcaccatcagcagcctgcagcctgaagattttgcaacttattactgtctacaagatttcaattacccgtggcacttcggccaagggaccaaggtggaaatcaaa

SEQ ID NO: 130 - protein, 107 aa, synthetic construct
  REGION 1..107: note = synthetic
AIQMTQSPSSLSASVGDRVTITCRASQGIRNDLGWYQQKPGKAPKLLIYAASSLQSGVPSRFAGRGSGTDFTLTISSLQPEDFATYYCLQDFNYPWHFGQGTKVEIK

SEQ ID NO: 131 - DNA, 18 bp, synthetic construct
  misc_feature 1..18: note = synthetic
  source 1..18: mol_type = other DNA
cagggcattagaaatgat

SEQ ID NO: 132 - protein, 6 aa, synthetic construct
  REGION 1..6: note = synthetic
QGIRND

SEQ ID NO: 133-134 - skipped (2 entries)

SEQ ID NO: 135 - DNA, 27 bp, synthetic construct
  misc_feature 1..27: note = synthetic
  source 1..27: mol_type = other DNA
ctacaagatttcaattacccgtggcac

SEQ ID NO: 136 - protein, 9 aa, synthetic construct
  REGION 1..9: note = synthetic
LQDFNYPWH

SEQ ID NO: 137 - DNA, 360 bp, synthetic construct
  misc_feature 1..360: note = synthetic
  source 1..360: mol_type = other DNA
caggtgcagctgcaggagtcgggcccaggactggtgaagccttcggagaccctgtccctcacctgcactgtctctggtgactccgtcagtagttcctactggacctggatccggcagcccccagggaagggactggagtggattggctatatctattacagtgggagttccaactacaacccctccctcaagagtcgagccaccatttcagtagacacgtccaagaaccagttctccctgaagctgagttctgtgaccgctgcggacacggccgtatattactgtgcgagagaagggaacgtggatacaactatgatacatgactactggggccagggaaccctggtcaccgtctcctca

SEQ ID NO: 138 - protein, 120 aa, synthetic construct
  REGION 1..120: note = synthetic
QVQLQESGPGLVKPSETLSLTCTVSGDSVSSSYWTWIRQPPGKGLEWIGYIYYSGSSNYNPSLKSRATISVDTSKNQFSLKLSSVTAADTAVYYCAREGNVDTTMIHDYWGQGTLVTVSS

SEQ ID NO: 139 - DNA, 24 bp, synthetic construct
  misc_feature 1..24: note = synthetic
  source 1..24: mol_type = other DNA
ggtgactccgtcagtagttcctac

SEQ ID NO: 140 - protein, 8 aa, synthetic construct
  REGION 1..8: note = synthetic
GDSVSSSY

SEQ ID NO: 141 - DNA, 21 bp, synthetic construct
  misc_feature 1..21: note = synthetic
  source 1..21: mol_type = other DNA
atctattacagtgggagttcc

SEQ ID NO: 142 - protein, 7 aa, synthetic construct
  REGION 1..7: note = synthetic
IYYSGSS

SEQ ID NO: 143 - DNA, 42 bp, synthetic construct
  misc_feature 1..42: note = synthetic
  source 1..42: mol_type = other DNA
gcgagagaagggaacgtggatacaactatgatacatgactac

SEQ ID NO: 144 - protein, 14 aa, synthetic construct
  REGION 1..14: note = synthetic
AREGNVDTTMIHDY

SEQ ID NO: 145 - DNA, 360 bp, synthetic construct
  misc_feature 1..360: note = synthetic
  source 1..360: mol_type = other DNA
caggtgcagctgcaggagtcgggcccaggactggtgaagccttcggagaccctgtccctcacctgcactgtctctggtgactccgtcagtagttcctactggacctggatccggcagcccccagggaagggactggagtggattggctatatctattacagtgggagttccaactacaacccctccctcaagagtcgagccaccatttcagtagacacgtccaagaaccagttctccctgaagctgagttctgtgaccgctgcggacacggccgtatattactgtgcgagagaagggaacgtggatcacactatgatatttgactactggggccagggaaccctggtcaccgtctcctca

SEQ ID NO: 146 - protein, 120 aa, synthetic construct
  REGION 1..120: note = synthetic
QVQLQESGPGLVKPSETLSLTCTVSGDSVSSSYWTWIRQPPGKGLEWIGYIYYSGSSNYNPSLKSRATISVDTSKNQFSLKLSSVTAADTAVYYCAREGNVDHTMIFDYWGQGTLVTVSS

SEQ ID NO: 147 - DNA, 24 bp, synthetic construct
  misc_feature 1..24: note = synthetic
  source 1..24: mol_type = other DNA
ggtgactccgtcagtagttcctac

SEQ ID NO: 148 - protein, 8 aa, synthetic construct
  REGION 1..8: note = synthetic
GDSVSSSY

SEQ ID NO: 149 - DNA, 21 bp, synthetic construct
  misc_feature 1..21: note = synthetic
  source 1..21: mol_type = other DNA
atctattacagtgggagttcc

SEQ ID NO: 150 - protein, 7 aa, synthetic construct
  REGION 1..7: note = synthetic
IYYSGSS

SEQ ID NO: 151 - DNA, 42 bp, synthetic construct
  misc_feature 1..42: note = synthetic
  source 1..42: mol_type = other DNA
gcgagagaagggaacgtggatcacactatgatatttgactac

SEQ ID NO: 152 - protein, 14 aa, synthetic construct
  REGION 1..14: note = synthetic
AREGNVDHTMIFDY

SEQ ID NO: 153 - DNA, 360 bp, synthetic construct
  misc_feature 1..360: note = synthetic
  source 1..360: mol_type = other DNA
caggtgcagctggtggagtctgggggaggcttggtcaagcctggagggtccctgagactctcctgtgcagcctctggattcaccttcagtgactcctacatgtcctggatccgtcaggctccagggaagggactagagtggatttcatacattggtagtagtggtaataccttttactacgcagactctgtgaagggccggttcaccatttccagagacaacgccaacaatttactgtatctgcaaatgaccagcctgagagccgaggacacggccgtgtattactgtgcgagagaagaaggcgatttttggagtgccgttgactcctggggccagggaaccctggtcaccgtctcctca

SEQ ID NO: 154 - protein, 120 aa, synthetic construct
  REGION 1..120: note = synthetic
QVQLVESGGGLVKPGGSLRLSCAASGFTFSDSYMSWIRQAPGKGLEWISYIGSSGNTFYYADSVKGRFTISRDNANNLLYLQMTSLRAEDTAVYYCAREEGDFWSAVDSWGQGTLVTVSS

SEQ ID NO: 155 - DNA, 24 bp, synthetic construct
  misc_feature 1..24: note = synthetic
  source 1..24: mol_type = other DNA
ggattcaccttcagtgactcctac

SEQ ID NO: 156 - protein, 8 aa, synthetic construct
  REGION 1..8: note = synthetic
GFTFSDSY

SEQ ID NO: 157 - DNA, 24 bp, synthetic construct
  misc_feature 1..24: note = synthetic
  source 1..24: mol_type = other DNA
attggtagtagtggtaataccttt

SEQ ID NO: 158 - protein, 8 aa, synthetic construct
  REGION 1..8: note = synthetic
IGSSGNTF

SEQ ID NO: 159 - DNA, 39 bp, synthetic construct
  misc_feature 1..39: note = synthetic
  source 1..39: mol_type = other DNA
gcgagagaagaaggcgatttttggagtgccgttgactcc

SEQ ID NO: 160 - protein, 13 aa, synthetic construct
  REGION 1..13: note = synthetic
AREEGDFWSAVDS

SEQ ID NO: 161 - DNA, 321 bp, synthetic construct
  misc_feature 1..321: note = synthetic
  source 1..321: mol_type = other DNA
gacatccagttgacccagtctccatccttcctgtctgcatctgtaggagacagagtcaccatcacttgctgggccagtcagggcattagcagttatttagcctggtatcagcaaaaaccaggtaaagcccctaaactcctgatccatactgcatccactttgcaaagtggggtcccatcaaggttcagcggcagtggatctgggacagaattcactctcacaatcagcaacctgcagcctgaagattttgcaacttattactgtcaacagcttaatagttacccattcactttcggccctgggaccaaagtggatatcaaa

SEQ ID NO: 162 - protein, 107 aa, synthetic construct
  REGION 1..107: note = synthetic
DIQLTQSPSFLSASVGDRVTITCWASQGISSYLAWYQQKPGKAPKLLIHTASTLQSGVPSRFSGSGSGTEFTLTISNLQPEDFATYYCQQLNSYPFTFGPGTKVDIK

SEQ ID NO: 163 - DNA, 18 bp, synthetic construct
  misc_feature 1..18: note = synthetic
  source 1..18: mol_type = other DNA
cagggcattagcagttat

SEQ ID NO: 164 - protein, 6 aa, synthetic construct
  REGION 1..6: note = synthetic
QGISSY

SEQ ID NO: 165-166 - skipped (2 entries)

SEQ ID NO: 167 - DNA, 27 bp, synthetic construct
  misc_feature 1..27: note = synthetic
  source 1..27: mol_type = other DNA
caacagcttaatagttacccattcact

SEQ ID NO: 168 - protein, 9 aa, synthetic construct
  REGION 1..9: note = synthetic
QQLNSYPFT

SEQ ID NO: 169 - DNA, 366 bp, synthetic construct
  misc_feature 1..366: note = synthetic
  source 1..366: mol_type = other DNA
caggtgcagctggtggagtctgggggaggcgtggtccagcctggggggtccctgagactctcctgtgcagcctctggattcaccttcggtggccatgccatgcactgggtccgccaggctccaggcaaggggctggagtggctggcagttatatcatctgatggcagtaataaacagtatgcagattctgtgaagggccgattcaccatctccagggacaatcccaagaacacgctgtatctgcaaatgaacagtctgagagttggggacacggctatttattactgtgcgaaagaggtggcacctcgttattattattacggtctggacgtctggggccaagggaccacggtcaccgtctcctca

SEQ ID NO: 170 - protein, 122 aa, synthetic construct
  REGION 1..122: note = synthetic
QVQLVESGGGVVQPGGSLRLSCAASGFTFGGHAMHWVRQAPGKGLEWLAVISSDGSNKQYADSVKGRFTISRDNPKNTLYLQMNSLRVGDTAIYYCAKEVAPRYYYYGLDVWGQGTTVTVSS

SEQ ID NO: 171 - DNA, 24 bp, synthetic construct
  misc_feature 1..24: note = synthetic
  source 1..24: mol_type = other DNA
ggattcaccttcggtggccatgcc

SEQ ID NO: 172 - protein, 8 aa, synthetic construct
  REGION 1..8: note = synthetic
GFTFGGHA

SEQ ID NO: 173 - DNA, 24 bp, synthetic construct
  misc_feature 1..24: note = synthetic
  source 1..24: mol_type = other DNA
atatcatctgatggcagtaataaa

SEQ ID NO: 174 - protein, 8 aa, synthetic construct
  REGION 1..8: note = synthetic
ISSDGSNK

SEQ ID NO: 175 - DNA, 45 bp, synthetic construct
  misc_feature 1..45: note = synthetic
  source 1..45: mol_type = other DNA
gcgaaagaggtggcacctcgttattattattacggtctggacgtc

SEQ ID NO: 176 - protein, 15 aa, synthetic construct
  REGION 1..15: note = synthetic
AKEVAPRYYYYGLDV

SEQ ID NO: 177 - DNA, 318 bp, synthetic construct
  misc_feature 1..318: note = synthetic
  source 1..318: mol_type = other DNA
gacatccagatgacccagtctccatcctccctgtctgcatctgtgggagacagagtcaccatcacttgccgggcgagtcaggacattagcaattttttagcctggtatcagcagaaaccagggaaggttcctaaactcctgatctatactgcatccactttacaatcaggggtcccatctcggttcagtggcagtggatctgggacagatttcactctcaccgtcagcagcctacagcctgaagatgttgcaacttattactgtcaaaagtatgccggcgccctcactttcggccctgggaccaaagtggatatcaaa

SEQ ID NO: 178 - protein, 106 aa, synthetic construct
  REGION 1..106: note = synthetic
DIQMTQSPSSLSASVGDRVTITCRASQDISNFLAWYQQKPGKVPKLLIYTASTLQSGVPSRFSGSGSGTDFTLTVSSLQPEDVATYYCQKYAGALTFGPGTKVDIK

SEQ ID NO: 179 - DNA, 18 bp, synthetic construct
  misc_feature 1..18: note = synthetic
  source 1..18: mol_type = other DNA
caggacattagcaatttt

SEQ ID NO: 180 - protein, 6 aa, synthetic construct
  REGION 1..6: note = synthetic
QDISNF

SEQ ID NO: 181-182 - skipped (2 entries)

SEQ ID NO: 183 - DNA, 24 bp, synthetic construct
  misc_feature 1..24: note = synthetic
  source 1..24: mol_type = other DNA
caaaagtatgccggcgccctcact

SEQ ID NO: 184 - protein, 8 aa, synthetic construct
  REGION 1..8: note = synthetic
QKYAGALT

SEQ ID NO: 185 - DNA, 357 bp, synthetic construct
  misc_feature 1..357: note = synthetic
  source 1..357: mol_type = other DNA
gaggtgcagctggtggagtctgggggaggcttggcacagcctggggggtccctgagactctcctgtgcagcctctggattcacgtttagaagctatgccatgagctgggtccgccaggctccagggaaggggccggagtgggtctcaggtataggtggtaatggtgttaccacatactacgcagactccgtgaagggccggttcaccatctccagagacaattccaagaacacgctgtttctgcaaatgaatagcctgagagccgaggacacggccgtatattattgtgtgcaggggggtttaggtggttattttacaggctactggggccagggaaccctggtcaccgtctcctca

SEQ ID NO: 186 - protein, 119 aa, synthetic construct
  REGION 1..119: note = synthetic
EVQLVESGGGLAQPGGSLRLSCAASGFTFRSYAMSWVRQAPGKGPEWVSGIGGNGVTTYYADSVKGRFTISRDNSKNTLFLQMNSLRAEDTAVYYCVQGGLGGYFTGYWGQGTLVTVSS

SEQ ID NO: 187 - DNA, 24 bp, synthetic construct
  misc_feature 1..24: note = synthetic
  source 1..24: mol_type = other DNA
ggattcacgtttagaagctatgcc

SEQ ID NO: 188 - protein, 8 aa, synthetic construct
  REGION 1..8: note = synthetic
GFTFRSYA

SEQ ID NO: 189 - DNA, 24 bp, synthetic construct
  misc_feature 1..24: note = synthetic
  source 1..24: mol_type = other DNA
ataggtggtaatggtgttaccaca

SEQ ID NO: 190 - protein, 8 aa, synthetic construct
  REGION 1..8: note = synthetic
IGGNGVTT

SEQ ID NO: 191 - DNA, 36 bp, synthetic construct
  misc_feature 1..36: note = synthetic
  source 1..36: mol_type = other DNA
gtgcaggggggtttaggtggttattttacaggctac

SEQ ID NO: 192 - protein, 12 aa, synthetic construct
  REGION 1..12: note = synthetic
VQGGLGGYFTGY

SEQ ID NO: 193 - DNA, 321 bp, synthetic construct
  misc_feature 1..321: note = synthetic
  source 1..321: mol_type = other DNA
gacatccagatgacccagtctccatcctccctgtctgcatctgtaggagacagagtcaccatcacttgccgggcaagtcagagtattagtacctatttaaattggtatcagcagaatccagggaaagcccctaaactcctgatctttgatgcatccagtttgcaaagtggggtcccatcaaggttcagtggcagtggatctgggacagatttcactctcaccatcagaggtctgcaacctgaagattttgcaacttactactgtcaacagagttacagtgccccgctcactttcggcggagggaccaaggtggagatcaaa

SEQ ID NO: 194 - protein, 107 aa, synthetic construct
  REGION 1..107: note = synthetic
DIQMTQSPSSLSASVGDRVTITCRASQSISTYLNWYQQNPGKAPKLLIFDASSLQSGVPSRFSGSGSGTDFTLTIRGLQPEDFATYYCQQSYSAPLTFGGGTKVEIK

SEQ ID NO: 195 - DNA, 18 bp, synthetic construct
  misc_feature 1..18: note = synthetic
  source 1..18: mol_type = other DNA
cagagtattagtacctat

SEQ ID NO: 196 - protein, 6 aa, synthetic construct
  REGION 1..6: note = synthetic
QSISTY

SEQ ID NO: 197-198 - skipped (2 entries)

SEQ ID NO: 199 - DNA, 27 bp, synthetic construct
  misc_feature 1..27: note = synthetic
  source 1..27: mol_type = other DNA
caacagagttacagtgccccgctcact

SEQ ID NO: 200 - protein, 9 aa, synthetic construct
  REGION 1..9: note = synthetic
QQSYSAPLT

SEQ ID NO: 201 - DNA, 357 bp, synthetic construct
  misc_feature 1..357: note = synthetic
  source 1..357: mol_type = other DNA
caggtgcagctggtggagtctgggggaggcgtggtccagcctgggaggtccctgagactctcctgtgcagcgtctggattcaccttcagtggttatggcatgcactgggtccgccaggctccaggcaaggggctggagtgggtggcacttatatggcttgatggaagtaatgactactatgcagactccgtgaagggccgattcaccatctccagagacaattccaagaacacgttatatctgcaaatgaacagactgagagccgaggacacggctgtgtattactgtgcgagagatggcccggttgctgctatacccgactactggggccagggaaccctggtcaccgtctcctca

SEQ ID NO: 202 - protein, 119 aa, synthetic construct
  REGION 1..119: note = synthetic
QVQLVESGGGVVQPGRSLRLSCAASGFTFSGYGMHWVRQAPGKGLEWVALIWLDGSNDYYADSVKGRFTISRDNSKNTLYLQMNRLRAEDTAVYYCARDGPVAAIPDYWGQGTLVTVSS

SEQ ID NO: 203 - DNA, 24 bp, synthetic construct
  misc_feature 1..24: note = synthetic
  source 1..24: mol_type = other DNA
ggattcaccttcagtggttatggc

SEQ ID NO: 204 - protein, 8 aa, synthetic construct
  REGION 1..8: note = synthetic
GFTFSGYG

SEQ ID NO: 205 - DNA, 24 bp, synthetic construct
  misc_feature 1..24: note = synthetic
  source 1..24: mol_type = other DNA
atatggcttgatggaagtaatgac

SEQ ID NO: 206 - protein, 8 aa, synthetic construct
  REGION 1..8: note = synthetic
IWLDGSND

SEQ ID NO: 207 - DNA, 36 bp, synthetic construct
  misc_feature 1..36: note = synthetic
  source 1..36: mol_type = other DNA
gcgagagatggcccggttgctgctatacccgactac

SEQ ID NO: 208 - protein, 12 aa, synthetic construct
  REGION 1..12: note = synthetic
ARDGPVAAIPDY

SEQ ID NO: 209 - DNA, 321 bp, synthetic construct
  misc_feature 1..321: note = synthetic
  source 1..321: mol_type = other DNA
gacatccagatgacccagtctccttccaccctgtctgcatctgtaggagacagagtcaccatcacttgccgggccagtcagagtattagtaggtggttggcctggtatcagctgaaaccagggaaagcccctaagctcctgatctataaggcgtctagtttagaaagtggggtcccatcaaggttcagcggcagtggatctgggacagacttcactctcaccatcagcagcctgcaacctgatgattttgcaacttattactgccaacagtataatacttattcgtacacttttggccaggggaccaagctggagatcaaa

SEQ ID NO: 210 - protein, 107 aa, synthetic construct
  REGION 1..107: note = synthetic
DIQMTQSPSTLSASVGDRVTITCRASQSISRWLAWYQLKPGKAPKLLIYKASSLESGVPSRFSGSGSGTDFTLTISSLQPDDFATYYCQQYNTYSYTFGQGTKLEIK

SEQ ID NO: 211 - DNA, 18 bp, synthetic construct
  misc_feature 1..18: note = synthetic
  source 1..18: mol_type = other DNA
cagagtattagtaggtgg

SEQ ID NO: 212 - protein, 6 aa, synthetic construct
  REGION 1..6: note = synthetic
QSISRW

SEQ ID NO: 213-214 - skipped (2 entries)

SEQ ID NO: 215 - DNA, 27 bp, synthetic construct
  misc_feature 1..27: note = synthetic
  source 1..27: mol_type = other DNA
caacagtataatacttattcgtacact

SEQ ID NO: 216 - protein, 9 aa, synthetic construct
  REGION 1..9: note = synthetic
QQYNTYSYT

SEQ ID NO: 217 - DNA, 363 bp, synthetic construct
  misc_feature 1..363: note = synthetic
  source 1..363: mol_type = other DNA
gaggtgcagctggtggagtctgggggaggtgtggtacggcctggggggtccctgagactctcctgtgcagcctctggattcacctttgatgaatatggcatgacttgggtccgccaagttccagggaaggggctggagtgggtctctggtattacttggaatggtggtttcacagattatacagactctgtgaagggccgattcaccagctccagagacaacgccaagaactccctgtatctgcaaatgaacagtctgagagccgaggacacggccttgtattactgtgcgagagatggatatagcagctcgtggggggcttatgatatatggggccaagggacaatggtcaccgtctcttca

SEQ ID NO: 218 - protein, 121 aa, synthetic construct
  REGION 1..121: note = synthetic
EVQLVESGGGVVRPGGSLRLSCAASGFTFDEYGMTWVRQVPGKGLEWVSGITWNGGFTDYTDSVKGRFTSSRDNAKNSLYLQMNSLRAEDTALYYCARDGYSSSWGAYDIWGQGTMVTVSS

SEQ ID NO: 219 - DNA, 24 bp, synthetic construct
  misc_feature 1..24: note = synthetic
  source 1..24: mol_type = other DNA
ggattcacctttgatgaatatggc

SEQ ID NO: 220 - protein, 8 aa, synthetic construct
  REGION 1..8: note = synthetic
GFTFDEYG

SEQ ID NO: 221 - DNA, 24 bp, synthetic construct
  misc_feature 1..24: note = synthetic
  source 1..24: mol_type = other DNA
attacttggaatggtggtttcaca

SEQ ID NO: 222 - protein, 8 aa, synthetic construct
  REGION 1..8: note = synthetic
ITWNGGFT

SEQ ID NO: 223 - DNA, 42 bp, synthetic construct
  misc_feature 1..42: note = synthetic
  source 1..42: mol_type = other DNA
gcgagagatggatatagcagctcgtggggggcttatgatata

SEQ ID NO: 224 - protein, 14 aa, synthetic construct
  REGION 1..14: note = synthetic
ARDGYSSSWGAYDI

SEQ ID NO: 225 - DNA, 321 bp, synthetic construct
  misc_feature 1..321: note = synthetic
  source 1..321: mol_type = other DNA
gacatccagatgacccagtctccatcatccctgtctgcatctgtgggagacagagtcaccatcacttgccgggcaagtcagagcattagcacctatttaaattggtatcagcagaaaccagggaaagcccctaagctcctgatctatgctgcatccagtttgcaaagtggggtcccattaaggttcagtggcagtggatctgggactgatttcactctcaccatcagcagtctgcaacctgaagattttgcaagttatttctgtcaacagagttacagtaccccgtacacttttggccaggggaccaagctggagatcaaa

SEQ ID NO: 226 - protein, 107 aa, synthetic construct
  REGION 1..107: note = synthetic
DIQMTQSPSSLSASVGDRVTITCRASQSISTYLNWYQQKPGKAPKLLIYAASSLQSGVPLRFSGSGSGTDFTLTISSLQPEDFASYFCQQSYSTPYTFGQGTKLEIK

SEQ ID NO: 227 - DNA, 18 bp, synthetic construct
  misc_feature 1..18: note = synthetic
  source 1..18: mol_type = other DNA
cagagcattagcacctat

SEQ ID NO: 228 - protein, 6 aa, synthetic construct
  REGION 1..6: note = synthetic
QSISTY

SEQ ID NO: 229-230 - skipped (2 entries)

SEQ ID NO: 231 - DNA, 27 bp, synthetic construct
  misc_feature 1..27: note = synthetic
  source 1..27: mol_type = other DNA
caacagagttacagtaccccgtacact

SEQ ID NO: 232 - protein, 9 aa, synthetic construct
  REGION 1..9: note = synthetic
QQSYSTPYT

SEQ ID NO: 233 - DNA, 360 bp, synthetic construct
  misc_feature 1..360: note = synthetic
  source 1..360: mol_type = other DNA
gaagtgcagctggtggagtctgggggaggcgtggtacagcctggggggtccctgagactctcctgtgcagcctctggattcacctttaatgattatgccatgcactgggtccgtcaagctccagggaagggtctggagtgggtctctcttattagtggagatggtggtaacacatactatgcagactctgtgaagggccgactcaccatctccagagacaacagcaaaaactccctgtatctgcaaatgaacagtctgagaacagaggacaccgccttatattactgtgcaaaagataagggctggaacttcggttacttcgatctctggggccgtggcaccctggtcactgtctcctca

SEQ ID NO: 234 - protein, 120 aa, synthetic construct
  REGION 1..120: note = synthetic
EVQLVESGGGVVQPGGSLRLSCAASGFTFNDYAMHWVRQAPGKGLEWVSLISGDGGNTYYADSVKGRLTISRDNSKNSLYLQMNSLRTEDTALYYCAKDKGWNFGYFDLWGRGTLVTVSS

SEQ ID NO: 235 - DNA, 24 bp, synthetic construct
  misc_feature 1..24: note = synthetic
  source 1..24: mol_type = other DNA
ggattcacctttaatgattatgcc

SEQ ID NO: 236 - protein, 8 aa, synthetic construct
  REGION 1..8: note = synthetic
GFTFNDYA

SEQ ID NO: 237 - DNA, 24 bp, synthetic construct
  misc_feature 1..24: note = synthetic
  source 1..24: mol_type = other DNA
attagtggagatggtggtaacaca

SEQ ID NO: 238 - protein, 8 aa, synthetic construct
  REGION 1..8: note = synthetic
ISGDGGNT

SEQ ID NO: 239 - DNA, 39 bp, synthetic construct
  misc_feature 1..39: note = synthetic
  source 1..39: mol_type = other DNA
gcaaaagataagggctggaacttcggttacttcgatctc

SEQ ID NO: 240 - protein, 13 aa, synthetic construct
  REGION 1..13: note = synthetic
AKDKGWNFGYFDL

SEQ ID NO: 241 - DNA, 327 bp, synthetic construct
  misc_feature 1..327: note = synthetic
  source 1..327: mol_type = other DNA
gacatccagatgacccagtctccatcctccctgtctacatctgtgggagacagagtcaccatcacttgccgggcaagtcagaacattgacacctatttaaattggtatcagcagaaaccagggaaagcccctaaactcctgatctatgatgcatccagtttacaaagtggggtcccatcacggttcagtggcagcggatctgggacagatttcactctcaccatcaccagtctgcaacctgaagattttgccacttactactgtcaacagaatgacaatattcttcaccctctcactttcggcggagggaccaaggtggagatcaaa

SEQ ID NO: 242 - protein, 109 aa, synthetic construct
  REGION 1..109: note = synthetic
DIQMTQSPSSLSTSVGDRVTITCRASQNIDTYLNWYQQKPGKAPKLLIYDASSLQSGVPSRFSGSGSGTDFTLTITSLQPEDFATYYCQQNDNILHPLTFGGGTKVEIK

SEQ ID NO: 243 - DNA, 18 bp, synthetic construct
  misc_feature 1..18: note = synthetic
  source 1..18: mol_type = other DNA
cagaacattgacacctat

SEQ ID NO: 244 - protein, 6 aa, synthetic construct
  REGION 1..6: note = synthetic
QNIDTY

SEQ ID NO: 245-246 - skipped (2 entries)

SEQ ID NO: 247 - DNA, 33 bp, synthetic construct
  misc_feature 1..33: note = synthetic
  source 1..33: mol_type = other DNA
caacagaatgacaatattcttcaccctctcact

SEQ ID NO: 248 - protein, 11 aa, synthetic construct
  REGION 1..11: note = synthetic
QQNDNILHPLT

SEQ ID NO: 249 - DNA, 369 bp, synthetic construct
  misc_feature 1..369: note = synthetic
  source 1..369: mol_type = other DNA
gaggtgcagctggtggagtctgggggaggcttggtccaaccgggggggtccctgagactctcctgtgcagcctctggattccactctaatagatattggatggactgggtccgccaggctccagggaaggggctggagtgggtggccaacataaagcaagatggaagtgaggaaaactatgtggactctgtgaagggccgattcaccatctccagagacaacgccaagaactcactttatctgcaaatgaacagcctgagagccgaggacacggctgtgtattactgtgcgagagatcgaagcacctcgtgggtcccttactggttcttcgatctctggggccgtggcaccctggtcactgtctcctca

SEQ ID NO: 250 - protein, 123 aa, synthetic construct
  REGION 1..123: note = synthetic
EVQLVESGGGLVQPGGSLRLSCAASGFHSNRYWMDWVRQAPGKGLEWVANIKQDGSEENYVDSVKGRFTISRDNAKNSLYLQMNSLRAEDTAVYYCARDRSTSWVPYWFFDLWGRGTLVTVSS

SEQ ID NO: 251 - DNA, 24 bp, synthetic construct
  misc_feature 1..24: note = synthetic
  source 1..24: mol_type = other DNA
ggattccactctaatagatattgg

SEQ ID NO: 252 - protein, 8 aa, synthetic construct
  REGION 1..8: note = synthetic
GFHSNRYW

SEQ ID NO: 253 - DNA, 24 bp, synthetic construct
  misc_feature 1..24: note = synthetic
  source 1..24: mol_type = other DNA
ataaagcaagatggaagtgaggaa

SEQ ID NO: 254 - protein, 8 aa, synthetic construct
  REGION 1..8: note = synthetic
IKQDGSEE

SEQ ID NO: 255 - DNA, 48 bp, synthetic construct
  misc_feature 1..48: note = synthetic
  source 1..48: mol_type = other DNA
gcgagagatcgaagcacctcgtgggtcccttactggttcttcgatctc

SEQ ID NO: 256 - protein, 16 aa, synthetic construct
  REGION 1..16: note = synthetic
ARDRSTSWVPYWFFDL

SEQ ID NO: 257 - DNA, 324 bp, synthetic construct
  misc_feature 1..324: note = synthetic
  source 1..324: mol_type = other DNA
gacatccagatgacccagtctccatcctccctgtctgcatctgtaggagacagagtcaccatcacttgccgggcaagtcagagcattagcagctatttaaattggtatcagcagaaaccagggaaagcccctaagctcctgatctatgctgcatccagtttgcaaagtggggtcccgtcaaggttcagtggcagtggatctgggacagatttcactctcaccatcagcagtctgcaacctgaagattttgcaacttactactgtcaacagagttacagtacccctccgatcaccttcggccaagggacacgactggagattaaa

SEQ ID NO: 258 - protein, 108 aa, synthetic construct
  REGION 1..108: note = synthetic
DIQMTQSPSSLSASVGDRVTITCRASQSISSYLNWYQQKPGKAPKLLIYAASSLQSGVPSRFSGSGSGTDFTLTISSLQPEDFATYYCQQSYSTPPITFGQGTRLEIK

SEQ ID NO: 259 - DNA, 18 bp, synthetic construct
  misc_feature 1..18: note = synthetic
  source 1..18: mol_type = other DNA
cagagcattagcagctat

SEQ ID NO: 260 - protein, 6 aa, synthetic construct
  REGION 1..6: note = synthetic
QSISSY

SEQ ID NO: 261-262 - skipped (2 entries)

SEQ ID NO: 263 - DNA, 30 bp, synthetic construct
  misc_feature 1..30: note = synthetic
  source 1..30: mol_type = other DNA
caacagagttacagtacccctccgatcacc

SEQ ID NO: 264 - protein, 10 aa, synthetic construct
  REGION 1..10: note = synthetic
QQSYSTPPIT

SEQ ID NO: 265 - DNA, 360 bp, synthetic construct
  misc_feature 1..360: note = synthetic
  source 1..360: mol_type = other DNA
gaagtgcagctggtggagtctgggggaggcgtggtacagcggggggagtccctgagactctcctgttcagcctctgacttcatctttaaagattatgccatgtactgggtccgtcaaattccagggaagggtctagagtggatctctcttattagtggtgatggtgacactacatggtatggagactctgtgaagggccgattcaccatctccagagacaacaacgaaaactccctctttctgcaaatgaacgatctgagaactgaggacaccgccatgtactactgtgcaagagatatggggtggaacttctttcagttgcaatactggggccagggaaccctggtcaccgtctcctca

SEQ ID NO: 266 - protein, 120 aa, synthetic construct
  REGION 1..120: note = synthetic
EVQLVESGGGVVQRGESLRLSCSASDFIFKDYAMYWVRQIPGKGLEWISLISGDGDTTWYGDSVKGRFTISRDNNENSLFLQMNDLRTEDTAMYYCARDMGWNFFQLQYWGQGTLVTVSS

SEQ ID NO: 267 - DNA, 24 bp, synthetic construct
  misc_feature 1..24: note = synthetic
  source 1..24: mol_type = other DNA
gacttcatctttaaagattatgcc

SEQ ID NO: 268 - protein, 8 aa, synthetic construct
  REGION 1..8: note = synthetic
DFIFKDYA

SEQ ID NO: 269 - DNA, 24 bp, synthetic construct
  misc_feature 1..24: note = synthetic
  source 1..24: mol_type = other DNA
attagtggtgatggtgacactaca

SEQ ID NO: 270 - protein, 8 aa, synthetic construct
  REGION 1..8: note = synthetic
ISGDGDTT

SEQ ID NO: 271 - DNA, 39 bp, synthetic construct
  misc_feature 1..39: note = synthetic
  source 1..39: mol_type = other DNA
gcaagagatatggggtggaacttctttcagttgcaatac

SEQ ID NO: 272 - protein, 13 aa, synthetic construct
  REGION 1..13: note = synthetic
ARDMGWNFFQLQY

SEQ ID NO: 273 - DNA, 361 bp, synthetic construct
  misc_feature 1..361: note = synthetic
  source 1..361: mol_type = other DNA
dcaggtgcagctgcaggagtcgggccccgcactggtgaagccttcacagaccctgtccctcacctgcactgtctctggtggctccatcatcagaggtagtacctactggagttgggtccgccaattcccagggaagggcctggagtggattggatacagttattacagtgggaccgcctactataatccgtccctcgagagtcgagctaccatttctgtagacacgtctaagaaccagttctccctgaacctgaagtctgtgacggccgcggacacggccgtgtattattgtacaagagaaataggagtggctggtctctttgacatctggggccagggaaccctggtcaccgtctcctca

SEQ ID NO: 274 - protein, 120 aa, synthetic construct
  REGION 1..120: note = synthetic
QVQLQESGPALVKPSQTLSLTCTVSGGSIIRGSTYWSWVRQFPGKGLEWIGYSYYSGTAYYNPSLESRATISVDTSKNQFSLNLKSVTAADTAVYYCTREIGVAGLFDIWGQGTLVTVSS

SEQ ID NO: 275 - DNA, 30 bp, synthetic construct
  misc_feature 1..30: note = synthetic
  source 1..30: mol_type = other DNA
ggtggctccatcatcagaggtagtacctac

SEQ ID NO: 276 - protein, 10 aa, synthetic construct
  REGION 1..10: note = synthetic
GGSIIRGSTY

SEQ ID NO: 277 - DNA, 21 bp, synthetic construct
  misc_feature 1..21: note = synthetic
  source 1..21: mol_type = other DNA
agttattacagtgggaccgcc

SEQ ID NO: 278 - protein, 7 aa, synthetic construct
  REGION 1..7: note = synthetic
SYYSGTA

SEQ ID NO: 279 - DNA, 36 bp, synthetic construct
  misc_feature 1..36: note = synthetic
  source 1..36: mol_type = other DNA
acaagagaaataggagtggctggtctctttgacatc

SEQ ID NO: 280 - protein, 12 aa, synthetic construct
  REGION 1..12: note = synthetic
TREIGVAGLFDI

SEQ ID NO: 281 - DNA, 324 bp, synthetic construct
  misc_feature 1..324: note = synthetic
  source 1..324: mol_type = other DNA
gaaatagttttgacacagagtcccggcacactgtcactctctcccggggaaagagccaccttgtcatgtagagcaagtcagtcagtctctagctcttatctcgcctggtaccagcagaagccgggacaggcccctagactgctgatctacggggcaagttccagggccaccggaatccccgaccggttcagtggaagcggaagcggaaccgattttactttgacgatttctagactggagccagaggatttcgccgtttactattgtcaacagtacggaagcagcccgtggacgtttggccagggcacgaaggtagaaatcaag

SEQ ID NO: 282 - protein, 108 aa, synthetic construct
  REGION 1..108: note = synthetic
EIVLTQSPGTLSLSPGERATLSCRASQSVSSSYLAWYQQKPGQAPRLLIYGASSRATGIPDRFSGSGSGTDFTLTISRLEPEDFAVYYCQQYGSSPWTFGQGTKVEIK

SEQ ID NO: 283 - DNA, 36 bp, synthetic construct
  misc_feature 1..36: note = synthetic
  source 1..36: mol_type = other DNA
agagcaagtcagtcagtctctagctcttatctcgcc

SEQ ID NO: 284 - protein, 12 aa, synthetic construct
  REGION 1..12: note = synthetic
RASQSVSSSYLA

SEQ ID NO: 285 - DNA, 21 bp, synthetic construct
  misc_feature 1..21: note = synthetic
  source 1..21: mol_type = other DNA
ggggcaagttccagggccacc

SEQ ID NO: 286 - protein, 7 aa, synthetic construct
  REGION 1..7: note = synthetic
GASSRAT

SEQ ID NO: 287 - DNA, 27 bp, synthetic construct
  misc_feature 1..27: note = synthetic
  source 1..27: mol_type = other DNA
caacagtacggaagcagcccgtggacg

SEQ ID NO: 288 - protein, 9 aa, synthetic construct
  REGION 1..9: note = synthetic
QQYGSSPWT

SEQ ID NO: 289 - DNA, 357 bp, synthetic construct
  misc_feature 1..357: note = synthetic
  source 1..357: mol_type = other DNA
caggagcagttggtgcagtctggggctgaggtgaagaagcctggggcctcagtgaaggtctcctgtaaggcttctggatacaccttcaccggctactatatacattgggtgcgacaggcccctggactagggcttgaatggatgggatggatcaaccctaacagtggtggcacaaaatatgcacagaagtttcagggcagggtcaccatgaccagggacacgtccatcaatacagcctacatggagctgaaaagactgaaatctgacgactcggccgtatattactgtgcgagagacgcccctccccatgatgtttttgatatctggggccaagggacattggtcaccgtctcttca

SEQ ID NO: 290 - protein, 119 aa, synthetic construct
  REGION 1..119: note = synthetic
QEQLVQSGAEVKKPGASVKVSCKASGYTFTGYYIHWVRQAPGLGLEWMGWINPNSGGTKYAQKFQGRVTMTRDTSINTAYMELKRLKSDDSAVYYCARDAPPHDVFDIWGQGTLVTVSS

SEQ ID NO: 291 - DNA, 24 bp, synthetic construct
  misc_feature 1..24: note = synthetic
  source 1..24: mol_type = other DNA
ggatacaccttcaccggctactat

SEQ ID NO: 292 - protein, 8 aa, synthetic construct
  REGION 1..8: note = synthetic
GYTFTGYY

SEQ ID NO: 293 - DNA, 24 bp, synthetic construct
  misc_feature 1..24: note = synthetic
  source 1..24: mol_type = other DNA
atcaaccctaacagtggtggcaca

SEQ ID NO: 294 - protein, 8 aa, synthetic construct
  REGION 1..8: note = synthetic
INPNSGGT

SEQ ID NO: 295 - DNA, 36 bp, synthetic construct
  misc_feature 1..36: note = synthetic
  source 1..36: mol_type = other DNA
gcgagagacgcccctccccatgatgtttttgatatc

SEQ ID NO: 296 - protein, 12 aa, synthetic construct
  REGION 1..12: note = synthetic
ARDAPPHDVFDI

SEQ ID NO: 297 - DNA, 321 bp, synthetic construct
  misc_feature 1..321: note = synthetic
  source 1..321: mol_type = other DNA
gacatccagatgacccagtctccatcctccctgtctgcatctgtaggagacagagtcaccatcacttgccgggcaagtcagggcattagaaatgatttaggctggtatcagcagaaaccagggaaagcccctaagcgcctgatctatgctgcatccagtttgcaaattggggtcccatcaaggttcagcggcagtggatctgggacagaattcactctcacaatcagcagcctgcagcctgaagattttgcaacttattactgtctacagcataatagttacccgctcactttcggcggagggaccaaggtggagatcaaa

SEQ ID NO: 298 - protein, 107 aa, synthetic construct
  REGION 1..107: note = synthetic
DIQMTQSPSSLSASVGDRVTITCRASQGIRNDLGWYQQKPGKAPKRLIYAASSLQIGVPSRFSGSGSGTEFTLTISSLQPEDFATYYCLQHNSYPLTFGGGTKVEIK

SEQ ID NO: 299 - DNA, 18 bp, synthetic construct
  misc_feature 1..18: note = synthetic
  source 1..18: mol_type = other DNA
cagggcattagaaatgat

SEQ ID NO: 300 - protein, 6 aa, synthetic construct
  REGION 1..6: note = synthetic
QGIRND

SEQ ID NO: 301-302 - skipped (2 entries)

SEQ ID NO: 303 - DNA, 27 bp, synthetic construct
  misc_feature 1..27: note = synthetic
  source 1..27: mol_type = other DNA
ctacagcataatagttacccgctcact

SEQ ID NO: 304 - protein, 9 aa, synthetic construct
  REGION 1..9: note = synthetic
LQHNSYPLT

SEQ ID NO: 305 - DNA, 357 bp, synthetic construct
  misc_feature 1..357: note = synthetic
  source 1..357: mol_type = other DNA
caggtgcagctgcaagagtcgggcccaggactggtgaagccttcacagaccctgtccctcacctgcactgtctctggtggctccatcagtagtggtgcttaccactggagctggatccgccagcacccagggaagggcctagagtggattggatacatctattacaatggggacacctactataatccgtccctcaagagtcgcgttaccatttcagtggacacgtctaagaaccaattcttcctgaaggtgacctctgtgactgccgcggacacggccatgtattactgtgcgggagaaaagcagctgactgcttttgatatctggggccaagggacattggtcaccgtctcttca

SEQ ID NO: 306 - protein, 119 aa, synthetic construct
  REGION 1..119: note = synthetic
QVQLQESGPGLVKPSQTLSLTCTVSGGSISSGAYHWSWIRQHPGKGLEWIGYIYYNGDTYYNPSLKSRVTISVDTSKNQFFLKVTSVTAADTAMYYCAGEKQLTAFDIWGQGTLVTVSS

SEQ ID NO: 307 - DNA, 30 bp, synthetic construct
  misc_feature 1..30: note = synthetic
  source 1..30: mol_type = other DNA
ggtggctccatcagtagtggtgcttaccac

SEQ ID NO: 308 - protein, 10 aa, synthetic construct
  REGION 1..10: note = synthetic
GGSISSGAYH

SEQ ID NO: 309 - DNA, 21 bp, synthetic construct
  misc_feature 1..21: note = synthetic
  source 1..21: mol_type = other DNA
atctattacaatggggacacc

SEQ ID NO: 310 - protein, 7 aa, synthetic construct
  REGION 1..7: note = synthetic
IYYNGDT

SEQ ID NO: 311 - DNA, 33 bp, synthetic construct
  misc_feature 1..33: note = synthetic
  source 1..33: mol_type = other DNA
gcgggagaaaagcagctgactgcttttgatatc

SEQ ID NO: 312 - protein, 11 aa, synthetic construct
  REGION 1..11: note = synthetic
AGEKQLTAFDI

SEQ ID NO: 313 - DNA, 321 bp, synthetic construct
  misc_feature 1..321: note = synthetic
  source 1..321: mol_type = other DNA
gtcatccagatgacccagtctccatcctccctgtctgcatctgttggagacagagtcaccataacttgccgggcgagtcaggacattaataattttttaaattggtatcaacagaaattagggaaagcccctaaactcctgatctccgatgcatccaatttgcagacaggagtcccgtcaaggttcagtggaagtggatctgggacagattttactttcaccatcagcagcctgcagcctgaagatattgctgcatattactgtcaacaatatgatcatttcccgtatacttttggccaggggaccagactggagaacaat

SEQ ID NO: 314 - protein, 107 aa, synthetic construct
  REGION 1..107: note = synthetic
VIQMTQSPSSLSASVGDRVTITCRASQDINNFLNWYQQKLGKAPKLLISDASNLQTGVPSRFSGSGSGTDFTFTISSLQPEDIAAYYCQQYDHFPYTFGQGTRLENN

SEQ ID NO: 315 - DNA, 18 bp, synthetic construct
  misc_feature 1..18: note = synthetic
  source 1..18: mol_type = other DNA
caggacattaataatttt

SEQ ID NO: 316 - protein, 6 aa, synthetic construct
  REGION 1..6: note = synthetic
QDINNF

SEQ ID NO: 317-318 - skipped (2 entries)

SEQ ID NO: 319 - DNA, 27 bp, synthetic construct
  misc_feature 1..27: note = synthetic
  source 1..27: mol_type = other DNA
caacaatatgatcatttcccgtatact

SEQ ID NO: 320 - protein, 9 aa, synthetic construct
  REGION 1..9: note = synthetic
QQYDHFPYT

SEQ ID NO: 321 - DNA, 357 bp, synthetic construct
  misc_feature 1..357: note = synthetic
  source 1..357: mol_type = other DNA
gaggtgcagttggtggagtctgggggaggtgtggttcggcctggggggtccctgagactctcctgtgcagcctctggattcacctttgatgattatggcatgacctgggtccgccaagctccagggaaggggctggagtgggtctctggtattaattggaatggcgatagcacagagtattcagactctgtgaagggccgattcaccatctccagagacaacgccaagaactccctgtatctgcaaatgaacagtctgagagccgaggacacggccttctatcactgtgcgagagagaataactggaacttctactttgactactggggccagggaaccctggtcaccgtctcctca

SEQ ID NO: 322 - protein, 119 aa, synthetic construct
  REGION 1..119: note = synthetic
EVQLVESGGGVVRPGGSLRLSCAASGFTFDDYGMTWVRQAPGKGLEWVSGINWNGDSTEYSDSVKGRFTISRDNAKNSLYLQMNSLRAEDTAFYHCARENNWNFYFDYWGQGTLVTVSS

SEQ ID NO: 323 - DNA, 24 bp, synthetic construct
  misc_feature 1..24: note = synthetic
  source 1..24: mol_type = other DNA
ggattcacctttgatgattatggc

SEQ ID NO: 324 - protein, 8 aa, synthetic construct
  REGION 1..8: note = synthetic
GFTFDDYG

SEQ ID NO: 325 - DNA, 24 bp, synthetic construct
  misc_feature 1..24: note = synthetic
  source 1..24: mol_type = other DNA
attaattggaatggcgatagcaca

SEQ ID NO: 326 - protein, 8 aa, synthetic construct
  REGION 1..8: note = synthetic
INWNGDST

SEQ ID NO: 327 - DNA, 36 bp, synthetic construct
  misc_feature 1..36: note = synthetic
  source 1..36: mol_type = other DNA
gcgagagagaataactggaacttctactttgactac

SEQ ID NO: 328 - protein, 12 aa, synthetic construct
  REGION 1..12: note = synthetic
ARENNWNFYFDY

SEQ ID NO: 329 - DNA, 321 bp, synthetic construct
  misc_feature 1..321: note = synthetic
  source 1..321: mol_type = other DNA
gaaatagtgatgacgcagtctccagccaccctgtctgtgtctcgaggggaaagagccaccctctcctgtagggccagtcagagtgttagcagcaacttagcctggtaccagcagaaacttggccaggctcccaggctcctcatctatggtgcatccaccagggccactggtatcccagccaggttcagtggcagtgggtctgggacagagttcactctcaccatcagcagcctgcagtctgaagattttgcagtttattattgtcagcagtataataactggccgtggacgttcggccaagggaccaaggtggaaatcaaa

SEQ ID NO: 330 - protein, 107 aa, synthetic construct
  REGION 1..107: note = synthetic
EIVMTQSPATLSVSRGERATLSCRASQSVSSNLAWYQQKLGQAPRLLIYGASTRATGIPARFSGSGSGTEFTLTISSLQSEDFAVYYCQQYNNWPWTFGQGTKVEIK

SEQ ID NO: 331 - DNA, 18 bp, synthetic construct
  misc_feature 1..18: note = synthetic
  source 1..18: mol_type = other DNA
cagagtgttagcagcaac

SEQ ID NO: 332 - protein, 6 aa, synthetic construct
  REGION 1..6: note = synthetic
QSVSSN

SEQ ID NO: 333-334 - skipped (2 entries)

SEQ ID NO: 335 - DNA, 27 bp, synthetic construct
  misc_feature 1..27: note = synthetic
  source 1..27: mol_type = other DNA
cagcagtataataactggccgtggacg

SEQ ID NO: 336 - protein, 9 aa, synthetic construct
  REGION 1..9: note = synthetic
QQYNNWPWT

SEQ ID NO: 337 - DNA, 351 bp, synthetic construct
  misc_feature 1..351: note = synthetic
  source 1..351: mol_type = other DNA
caggtccacctggtacagtctggggctgaggtgaagaagcctggggcctcagtgaaggtctcctgcaaggtttccggaaacaccctcactgaattatccatgcactgggtgcgacaggctcctggaaaagggcttgagtggatgggaggttttgatcctgaagatggtgacacaatctactcacagaagttccagggcagagtcaccttgaccgaggacacatctacagacacagcctacatggagctgagcagcctgagatctgaggacacggccgtgtattactgttcaacagtggggggacctacctctgactgctggggccagggaaccctggtcaccgtctcctca

SEQ ID NO: 338 - protein, 117 aa, synthetic construct
  REGION 1..117: note = synthetic
QVHLVQSGAEVKKPGASVKVSCKVSGNTLTELSMHWVRQAPGKGLEWMGGFDPEDGDTIYSQKFQGRVTLTEDTSTDTAYMELSSLRSEDTAVYYCSTVGGPTSDCWGQGTLVTVSS

SEQ ID NO: 339 - DNA, 24 bp, synthetic construct
  misc_feature 1..24: note = synthetic
  source 1..24: mol_type = other DNA
ggaaacaccctcactgaattatcc

SEQ ID NO: 340 - protein, 8 aa, synthetic construct
  REGION 1..8: note = synthetic
GNTLTELS

SEQ ID NO: 341 - DNA, 24 bp, synthetic construct
  misc_feature 1..24: note = synthetic
  source 1..24: mol_type = other DNA
tttgatcctgaagatggtgacaca

SEQ ID NO: 342 - protein, 8 aa, synthetic construct
  REGION 1..8: note = synthetic
FDPEDGDT

SEQ ID NO: 343 - DNA, 30 bp, synthetic construct
  misc_feature 1..30: note = synthetic
  source 1..30: mol_type = other DNA
tcaacagtggggggacctacctctgactgc

SEQ ID NO: 344 - protein, 10 aa, synthetic construct
  REGION 1..10: note = synthetic
STVGGPTSDC

SEQ ID NO: 345 - DNA, 321 bp, synthetic construct
  misc_feature 1..321: note = synthetic
  source 1..321: mol_type = other DNA
gacatccagatgacccagtctccatcctccctgtctgcatctgtaggagacagagtcaccatcacttgccaggcgagtcaggacattagcaactatttaaattggtatcagcagaaaccagggaaagcccctaaggtcctgatcttcgatgcatccaatttagaaccaggggtcccatcaaggttcagtggaagtggatctgggacagattttactttcaccatcatcagcctgcagcctgaagatattgcaacatattactgtcaacaatatgataatctcccgatcaccttcggccaggggacacgactggacattaaa

SEQ ID NO: 346 - protein, 107 aa, synthetic construct
  REGION 1..107: note = synthetic
DIQMTQSPSSLSASVGDRVTITCQASQDISNYLNWYQQKPGKAPKVLIFDASNLEPGVPSRFSGSGSGTDFTFTIISLQPEDIATYYCQQYDNLPITFGQGTRLDIK

SEQ ID NO: 347 - DNA, 18 bp, synthetic construct
  misc_feature 1..18: note = synthetic
  source 1..18: mol_type = other DNA
caggacattagcaactat

SEQ ID NO: 348 - protein, 6 aa, synthetic construct
  REGION 1..6: note = synthetic
QDISNY

SEQ ID NO: 349-350 - skipped (2 entries)

SEQ ID NO: 351 - DNA, 27 bp, synthetic construct
  misc_feature 1..27: note = synthetic
  source 1..27: mol_type = other DNA
caacaatatgataatctcccgatcacc

SEQ ID NO: 352 - protein, 9 aa, synthetic construct
  REGION 1..9: note = synthetic
QQYDNLPIT

SEQ ID NO: 353 - protein, 447 aa, synthetic construct
  REGION 1..447: note = HC
QVQLQESGPGLVKPSETLSLTCTVSGDSVSSSYWTWIRQPPGKGLEWIGYIYYSGSSNYNPSLKSRATISVDTSKNQFSLKLSSVTAADTAVYYCAREGNVDTTMIFDYWGQGTLVTVSSASTKGPSVFPLAPCSRSTSESTAALGCLVKDYFPEPVTVSWNSGALTSGVHTFPAVLQSSGLYSLSSVVTVPSSSLGTKTYTCNVDHKPSNTKVDKRVESKYGPPCPPCPAPEFLGGPSVFLFPPKPKDTLMISRTPEVTCVVVDVSQEDPEVQFNWYVDGVEVHNAKTKPREEQFNSTYRVVSVLTVLHQDWLNGKEYKCKVSNKGLPSSIEKTISKAKGQPREPQVYTLPPSQEEMTKNQVSLTCLVKGFYPSDIAVEWESNGQPENNYKTTPPVLDSDGSFFLYSRLTVDKSRWQEGNVFSCSVMHEALHNHYTQKSLSLSLGK

SEQ ID NO: 354 - protein, 214 aa, synthetic construct
  REGION 1..214: note = LC
AIQMTQSPSSLSASVGDRVTITCRASQGIRNDLGWYQQKPGKAPKLLIYAASSLQSGVPSRFAGRGSGTDFTLTISSLQPEDFATYYCLQDFNYPWTFGQGTKVEIKRTVAAPSVFIFPPSDEQLKSGTASVVCLLNNFYPREAKVQWKVDNALQSGNSQESVTEQDSKDSTYSLSSTLTLSKADYEKHKVYACEVTHQGLSSPVTKSFNRGEC

SEQ ID NO: 355 - protein, 1676 aa, synthetic construct
  REGION 1..1676: note = human C5
MGLLGILCFLIFLGKTWGQEQTYVISAPKIFRVGASENIVIQVYGYTEAFDATISIKSYPDKKFSYSSGHVHLSSENKFQNSAILTIQPKQLPGGQNPVSYVYLEVVSKHFSKSKRMPITYDNGFLFIHTDKPVYTPDQSVKVRVYSLNDDLKPAKRETVLTFIDPEGSEVDMVEEIDHIGIISFPDFKIPSNPRYGMWTIKAKYKEDFSTTGTAYFEVKEYVLPHFSVSIEPEYNFIGYKNFKNFEITIKARYFYNKVVTEADVYITFGIREDLKDDQKEMMQTAMQNTMLINGIAQVTFDSETAVKELSYYSLEDLNNKYLYIAVTVIESTGGFSEEAEIPGIKYVLSPYKLNLVATPLFLKPGIPYPIKVQVKDSLDQLVGGVPVTLNAQTIDVNQETSDLDPSKSVTRVDDGVASFVLNLPSGVTVLEFNVKTDAPDLPEENQAREGYRAIAYSSLSQSYLYIDWTDNHKALLVGEHLNIIVTPKSPYIDKITHYNYLILSKGKIIHFGTREKFSDASYQSINIPVTQNMVPSSRLLVYYIVTGEQTAELVSDSVWLNIEEKCGNQLQVHLSPDADAYSPGQTVSLNMATGMDSWVALAAVDSAVYGVQRGAKKPLERVFQFLEKSDLGCGAGGGLNNANVFHLAGLTFLTNANADDSQENDEPCKEILRPRRTLQKKIEEIAAKYKHSVVKKCCYDGACVNNDETCEQRAARISLGPRCIKAFTECCVVASQLRANISHKDMQLGRLHMKTLLPVSKPEIRSYFPESWLWEVHLVPRRKQLQFALPDSLTTWEIQGVGISNTGICVADTVKAKVFKDVFLEMNIPYSVVRGEQIQLKGTVYNYRTSGMQFCVKMSAVEGICTSESPVIDHQGTKSSKCVRQKVEGSSSHLVTFTVLPLEIGLHNINFSLETWFGKEILVKTLRVVPEGVKRESYSGVTLDPRGIYGTISRRKEFPYRIPLDLVPKTEIKRILSVKGLLVGEILSAVLSQEGINILTHLPKGSAEAELMSVVPVFYVFHYLETGNHWNIFHSDPLIEKQKLKKKLKEGMLSIMSYRNADYSYSVWKGGSASTWLTAFALRVLGQVNKYVEQNQNSICNSLLWLVENYQLDNGSFKENSQYQPIKLQGTLPVEARENSLYLTAFTVIGIRKAFDICPLVKIDTALIKADNFLLENTLPAQSTFTLAISAYALSLGDKTHPQFRSIVSALKREALVKGNPPIYRFWKDNLQHKDSSVPNTGTARMVETTAYALLTSLNLKDINYVNPVIKWLSEEQRYGGGFYSTQDTINAIEGLTEYSLLVKQLRLSMDIDVSYKHKGALHNYKMTDKNFLGRPVEVLLNDDLIVSTGFGSGLATVHVTTVVHKTSTSEEVCSFYLKIDTQDIEASHYRGYGNSDYKRIVACASYKPSREESSSGSSHAVMDISLPTGISANEEDLKALVEGVDQLFTDYQIKDGHVILQLNSIPSSDFLCVRFRIFELFEVGFLSPATFTVYEYHRPDKQCTMFYSTSNIKIQKVCEGAACKCVEADCGQMQEELDLTISAETRKQTACKPEIAYAYKVSITSITVENVFVKYKATLLDIYKTGEAVAEKDSEITFIKKVTCTNAELVKGRQYLIMGKEALQIKYNFSFRYIYPLDSLTWIEYWPRDTTCSSCQAFLANLDEFAEDIFLNGC

SEQ ID NO: 356 - protein, 1686 aa, synthetic construct
  REGION 1..1686: note = hC5 R885H aa 1-1658: hC5 (aa 19-1676 of NM_001735.2 with R885H change) aa 1659-1686: myc-myc-hexahistidine tag
QEQTYVISAPKIFRVGASENIVIQVYGYTEAFDATISIKSYPDKKFSYSSGHVHLSSENKFQNSAILTIQPKQLPGGQNPVSYVYLEVVSKHFSKSKRMPITYDNGFLFIHTDKPVYTPDQSVKVRVYSLNDDLKPAKRETVLTFIDPEGSEVDMVEEIDHIGIISFPDFKIPSNPRYGMWTIKAKYKEDFSTTGTAYFEVKEYVLPHFSVSIEPEYNFIGYKNFKNFEITIKARYFYNKVVTEADVYITFGIREDLKDDQKEMMQTAMQNTMLINGIAQVTFDSETAVKELSYYSLEDLNNKYLYIAVTVIESTGGFSEEAEIPGIKYVLSPYKLNLVATPLFLKPGIPYPIKVQVKDSLDQLVGGVPVTLNAQTIDVNQETSDLDPSKSVTRVDDGVASFVLNLPSGVTVLEFNVKTDAPDLPEENQAREGYRAIAYSSLSQSYLYIDWTDNHKALLVGEHLNIIVTPKSPYIDKITHYNYLILSKGKIIHFGTREKFSDASYQSINIPVTQNMVPSSRLLVYYIVTGEQTAELVSDSVWLNIEEKCGNQLQVHLSPDADAYSPGQTVSLNMATGMDSWVALAAVDSAVYGVQRGAKKPLERVFQFLEKSDLGCGAGGGLNNANVFHLAGLTFLTNANADDSQENDEPCKEILRPRRTLQKKIEEIAAKYKHSVVKKCCYDGACVNNDETCEQRAARISLGPRCIKAFTECCVVASQLRANISHKDMQLGRLHMKTLLPVSKPEIRSYFPESWLWEVHLVPRRKQLQFALPDSLTTWEIQGVGISNTGICVADTVKAKVFKDVFLEMNIPYSVVRGEQIQLKGTVYNYRTSGMQFCVKMSAVEGICTSESPVIDHQGTKSSKCVHQKVEGSSSHLVTFTVLPLEIGLHNINFSLETWFGKEILVKTLRVVPEGVKRESYSGVTLDPRGIYGTISRRKEFPYRIPLDLVPKTEIKRILSVKGLLVGEILSAVLSQEGINILTHLPKGSAEAELMSVVPVFYVFHYLETGNHWNIFHSDPLIEKQKLKKKLKEGMLSIMSYRNADYSYSVWKGGSASTWLTAFALRVLGQVNKYVEQNQNSICNSLLWLVENYQLDNGSFKENSQYQPIKLQGTLPVEARENSLYLTAFTVIGIRKAFDICPLVKIDTALIKADNFLLENTLPAQSTFTLAISAYALSLGDKTHPQFRSIVSALKREALVKGNPPIYRFWKDNLQHKDSSVPNTGTARMVETTAYALLTSLNLKDINYVNPVIKWLSEEQRYGGGFYSTQDTINAIEGLTEYSLLVKQLRLSMDIDVSYKHKGALHNYKMTDKNFLGRPVEVLLNDDLIVSTGFGSGLATVHVTTVVHKTSTSEEVCSFYLKIDTQDIEASHYRGYGNSDYKRIVACASYKPSREESSSGSSHAVMDISLPTGISANEEDLKALVEGVDQLFTDYQIKDGHVILQLNSIPSSDFLCVRFRIFELFEVGFLSPATFTVYEYHRPDKQCTMFYSTSNIKIQKVCEGAACKCVEADCGQMQEELDLTISAETRKQTACKPEIAYAYKVSITSITVENVFVKYKATLLDIYKTGEAVAEKDSEITFIKKVTCTNAELVKGRQYLIMGKEALQIKYNFSFRYIYPLDSLTWIEYWPRDTTCSSCQAFLANLDEFAEDIFLNGCEQKLISEEDLGGEQKLISEEDLHHHHHH

SEQ ID NO: 357 - protein, 1686 aa, synthetic construct
  REGION 1..1686: note = hC5 R885C aa 1-1658: hC5 (aa 19-1676 of NM_001735.2 with R885C change) aa 1659-1686: myc-myc-hexahistidine tag
QEQTYVISAPKIFRVGASENIVIQVYGYTEAFDATISIKSYPDKKFSYSSGHVHLSSENKFQNSAILTIQPKQLPGGQNPVSYVYLEVVSKHFSKSKRMPITYDNGFLFIHTDKPVYTPDQSVKVRVYSLNDDLKPAKRETVLTFIDPEGSEVDMVEEIDHIGIISFPDFKIPSNPRYGMWTIKAKYKEDFSTTGTAYFEVKEYVLPHFSVSIEPEYNFIGYKNFKNFEITIKARYFYNKVVTEADVYITFGIREDLKDDQKEMMQTAMQNTMLINGIAQVTFDSETAVKELSYYSLEDLNNKYLYIAVTVIESTGGFSEEAEIPGIKYVLSPYKLNLVATPLFLKPGIPYPIKVQVKDSLDQLVGGVPVTLNAQTIDVNQETSDLDPSKSVTRVDDGVASFVLNLPSGVTVLEFNVKTDAPDLPEENQAREGYRAIAYSSLSQSYLYIDWTDNHKALLVGEHLNIIVTPKSPYIDKITHYNYLILSKGKIIHFGTREKFSDASYQSINIPVTQNMVPSSRLLVYYIVTGEQTAELVSDSVWLNIEEKCGNQLQVHLSPDADAYSPGQTVSLNMATGMDSWVALAAVDSAVYGVQRGAKKPLERVFQFLEKSDLGCGAGGGLNNANVFHLAGLTFLTNANADDSQENDEPCKEILRPRRTLQKKIEEIAAKYKHSVVKKCCYDGACVNNDETCEQRAARISLGPRCIKAFTECCVVASQLRANISHKDMQLGRLHMKTLLPVSKPEIRSYFPESWLWEVHLVPRRKQLQFALPDSLTTWEIQGVGISNTGICVADTVKAKVFKDVFLEMNIPYSVVRGEQIQLKGTVYNYRTSGMQFCVKMSAVEGICTSESPVIDHQGTKSSKCVCQKVEGSSSHLVTFTVLPLEIGLHNINFSLETWFGKEILVKTLRVVPEGVKRESYSGVTLDPRGIYGTISRRKEFPYRIPLDLVPKTEIKRILSVKGLLVGEILSAVLSQEGINILTHLPKGSAEAELMSVVPVFYVFHYLETGNHWNIFHSDPLIEKQKLKKKLKEGMLSIMSYRNADYSYSVWKGGSASTWLTAFALRVLGQVNKYVEQNQNSICNSLLWLVENYQLDNGSFKENSQYQPIKLQGTLPVEARENSLYLTAFTVIGIRKAFDICPLVKIDTALIKADNFLLENTLPAQSTFTLAISAYALSLGDKTHPQFRSIVSALKREALVKGNPPIYRFWKDNLQHKDSSVPNTGTARMVETTAYALLTSLNLKDINYVNPVIKWLSEEQRYGGGFYSTQDTINAIEGLTEYSLLVKQLRLSMDIDVSYKHKGALHNYKMTDKNFLGRPVEVLLNDDLIVSTGFGSGLATVHVTTVVHKTSTSEEVCSFYLKIDTQDIEASHYRGYGNSDYKRIVACASYKPSREESSSGSSHAVMDISLPTGISANEEDLKALVEGVDQLFTDYQIKDGHVILQLNSIPSSDFLCVRFRIFELFEVGFLSPATFTVYEYHRPDKQCTMFYSTSNIKIQKVCEGAACKCVEADCGQMQEELDLTISAETRKQTACKPEIAYAYKVSITSITVENVFVKYKATLLDIYKTGEAVAEKDSEITFIKKVTCTNAELVKGRQYLIMGKEALQIKYNFSFRYIYPLDSLTWIEYWPRDTTCSSCQAFLANLDEFAEDIFLNGCEQKLISEEDLGGEQKLISEEDLHHHHHH

SEQ ID NO: 358 - protein, 1686 aa, synthetic construct
  REGION 1..1686: note = M. fascicularis C5 R885H aa 1-1658: M. fascicularis C5 (determined in-house; NTBK#12480) aa 1659-1686: myc-myc-hexahistidine tag
QEQTYVISAPKIFRVGASENIVIQVYGYTEAFDATISIKSYPDKKFSYSSGHVHLSSENKFQNSAVLTIQPKQLPGGQNQVSYVYLEVVSKHFSKSKKIPITYDNGFLFIHTDKPVYTPDQSVKVRVYSLNDDLKPAKRETVLTFIDPEGSEIDMVEEIDHIGIISFPDFKIPSNPRYGMWTIQAKYKEDFSTTGTAFFEVKEYVLPHFSVSVEPESNFIGYKNFKNFEITIKARYFYNKVVTEADVYITFGIREDLKDDQKEMMQTAMQNTMLINGIAQVTFDSETAVKELSYYSLEDLNNKYLYIAVTVIESTGGFSEEAEIPGIKYVLSPYKLNLVATPLFLKPGIPYSIKVQVKDALDQLVGGVPVTLNAQTIDVNQETSDLEPRKSVTRVDDGVASFVVNLPSGVTVLEFNVKTDAPDLPDENQAREGYRAIAYSSLSQSYLYIDWTDNHKALLVGEYLNIIVTPKSPYIDKITHYNYLILSKGKIIHFGTREKLSDASYQSINIPVTQNMVPSSRLLVYYIVTGEQTAELVSDSVWLNIEEKCGNQLQVHLSPDADTYSPGQTVSLNMVTGMDSWVALTAVDSAVYGVQRRAKKPLERVFQFLEKSDLGCGAGGGLNNANVFHLAGLTFLTNANADDSQENDEPCKEIIRPRRMLQEKIEEIAAKYKHLVVKKCCYDGVRINHDETCEQRAARISVGPRCVKAFTECCVVASQLRANNSHKDLQLGRLHMKTLLPVSKPEIRSYFPESWLWEVHLVPRRKQLQFALPDSVTTWEIQGVGISNSGICVADTIKAKVFKDVFLEMNIPYSVVRGEQVQLKGTVYNYRTSGMQFCVKMSAVEGICTSESPVIDHQGTKSSKCVRQKVEGSSNHLVTFTVLPLEIGLQNINFSLETSFGKEILVKSLRVVPEGVKRESYSGITLDPRGIYGTISRRKEFPYRIPLDLVPKTEIKRILSVKGLLVGEILSAVLSREGINILTHLPKGSAEAELMSVVPVFYVFHYLETGNHWNIFHSDPLIEKRNLEKKLKEGMVSIMSYRNADYSYSVWKGGSASTWLTAFALRVLGQVHKHVEQNQNSICNSLLWLVENYQLDNGSFKENSQYQPIKLQGTLPVEARENSLYLTAFTVIGIRKAFDICPLVKINTALIKADTFLLENTLPAQSTFTLAISAYALSLGDKTHPQFRSIVSALKREALVKGNPPIYRFWKDSLQHKDSSVPNTGTARMVETTAYALLTSLNLKDINYVNPIIKWLSEEQRYGGGFYSTQDTINAIEGLTEYSLLVKQLRLNMDIDVAYKHKGPLHNYKMTDKNFLGRPVEVLLNDDLVVSTGFGSGLATVHVTTVVHKTSTSEEVCSFYLKIDTQDIEASHYRGYGNSDYKRIVACASYKPSREESSSGSSHAVMDISLPTGINANEEDLKALVEGVDQLFTDYQIKDGHVILQLNSIPSSDFLCVRFRIFELFEVGFLSPATFTVYEYHRPDKQCTMFYSTSNIKIQKVCEGATCKCIEADCGQMQKELDLTISAETRKQTACNPEIAYAYKVIITSITTENVFVKYKATLLDIYKTGEAVAEKDSEITFIKKVTCTNAELVKGRQYLIMGKEALQIKYNFTFRYIYPLDSLTWIEYWPRDTTCSSCQAFLANLDEFAEDIFLNGCEQKLISEEDLGGEQKLISEEDLHHHHHH

SEQ ID NO: 359 - protein, 1676 aa, synthetic construct; identical to SEQ ID NO: 355
  REGION 1..1676: note = hC5 P01031

SEQ ID NO: 360 - protein, 9 aa, synthetic construct
  REGION 1..9: note = human C5 peptide aa591-599
NMATGMDSW

SEQ ID NO: 361 - protein, 20 aa, synthetic construct
  REGION 1..20: note = human C5 peptide aa775-794
WEVHLVPRRKQLQFALPDSL

SEQ ID NO: 362 - protein, 121 aa, synthetic construct
  REGION 1..121: note = HCVR of M1M17628N
EVQLQESGPGLAKPSQTLSLTCSVTGYSITRDYWNWIRKFPGNKLDYMGYISYSGGTYYNPSLKSRFSISRDTSKNQFYLQLNSVTFEDTATYYCARGVSYYGSTYYFDYWGQGTTLTVSS

SEQ ID NO: 363 - protein, 107 aa, synthetic construct
  REGION 1..107: note = LCVR of M1M17628N
DIQMNQSPSSLSASLGDTITITCHASQNIHVWLNWYQQTPGNIPKLLIYKASNLHTGVPSRFSASGSGTGFTLTISSLQSEDIATYYCQQGQSYPLTFGGGTKLEIK

SEQ ID NO: 364 - protein, 20 aa, synthetic construct
  REGION 1..20: note = IRBP peptide
GPTHLFQPSLVLDMAKVLLD

SEQ ID NO: 365 - protein, 127 aa, synthetic construct
  REGION 1..127: note = HCVR of M1M17627N
QVQLQQPGAELVKPGASVKVSCKASGYTFTSYWIHWMRQRPGQGLEWIGRIHPSDSDTNYNQKFKGKATLTVDTSSSTAYMQLSSLTSEDSAVYYCAILPPPPYYYANYGGGTMDYWGRGTSVTVSS

SEQ ID NO: 366 - protein, 107 aa, synthetic construct
  REGION 1..107: note = LCVR of M1M17627N
DIVMTQSQKFMSTSVGDRVSVTCKASQNVGTNVVWYQQKPGQSPKALIYSASYRYSGVPARFTGSGSGTDFTLTITNVQSEDLAEYICQQYNRSPYTFGGGTKLETK